European Patent Specification EP 3 739 058 B1, published July 26, 2023. Title: Novel genes for regulating the virulence of Cryptococcus neoformans and their use. Applicant: YONSEI UNIVERSITY. The sequence listing filed with the application follows.

SEQUENCE LISTING (1380 sequences)

SEQ ID NO: 1 - DNA, 19 bp, CNAG_03132 5 flanking region primer 1
gcgtggcatttagagagtg

SEQ ID NO: 2 - DNA, 38 bp, CNAG_03132 5 flanking region primer 2
tcactggccgtcgttttacgagcgtattggatgaggag

SEQ ID NO: 3 - DNA, 39 bp, CNAG_03132 3 flanking region primer 1
catggtcatagctgtttcctgaaacctcgctttgagacg

SEQ ID NO: 4 - DNA, 18 bp, CNAG_03132 3 flanking region primer 2
tgacgaagcgacagaatc

SEQ ID NO: 5 - DNA, 20 bp, CNAG_03132 diagnostic screening primer, pairing with B79
cccaaacactattatcgcag

SEQ ID NO: 6 - DNA, 18 bp, CNAG_03132 Southern blot probe primer
tactcgtatgaatcggcg

SEQ ID NO: 7 - DNA, 20 bp, NAT#5 STM primer
tgctagagggcgggagagtt

SEQ ID NO: 8 - DNA, 24 bp, STM common primer
gcatgccctgcccctaagaattcg

SEQ ID NO: 9 - DNA, 20 bp, CNAG_05380 5 flanking region primer 1
cctactgcttggcacattac

SEQ ID NO: 10 - DNA, 35 bp, CNAG_05380 5 flanking region primer 2
ctggccgtcgttttaccgtcgtttctttttgggag

SEQ ID NO: 11 - DNA, 37 bp, CNAG_05380 3 flanking region primer 1
gtcatagctgtttcctgtccatctccagtctgtgaac

SEQ ID NO: 12 - DNA, 20 bp, CNAG_05380 3 flanking region primer 2
cgcttcttaggacctcactc

SEQ ID NO: 13 - DNA, 20 bp, CNAG_05380 diagnostic screening primer, pairing with B79
tctgaaggcggaatctggac

SEQ ID NO: 14 - DNA, 24 bp, CNAG_05380 Southern blot probe primer
ggagcaaggaactaaagatggtag

SEQ ID NO: 15 - DNA, 20 bp, NAT#5 STM primer
tgctagagggcgggagagtt

SEQ ID NO: 16 - DNA, 24 bp, STM common primer
gcatgccctgcccctaagaattcg

SEQ ID NO: 17 - DNA, 20 bp, CNAG_06719 5 flanking region primer 1
tcgccaactgaacaaacccc

SEQ ID NO: 18 - DNA, 36 bp, CNAG_06719 5 flanking region primer 2
ctggccgtcgttttactcccgcctaacactttcgtg

SEQ ID NO: 19 - DNA, 36 bp, CNAG_06719 3 flanking region primer 1
gtcatagctgtttcctgtgtcaagccataaagagcc

SEQ ID NO: 20 - DNA, 20 bp, CNAG_06719 3 flanking region primer 2
ctgatagttttgccacttgc

SEQ ID NO: 21 - DNA, 22 bp, CNAG_06719 diagnostic screening primer, pairing with B79
aataccctccttacttccccgc

SEQ ID NO: 22 - DNA, 18 bp, CNAG_06719 Southern blot probe primer
gtaaaagtttgggcgtgg

SEQ ID NO: 23 - DNA, 20 bp, NAT#5 STM primer
tgctagagggcgggagagtt

SEQ ID NO: 24 - DNA, 24 bp, STM common primer
gcatgccctgcccctaagaattcg

SEQ ID NO: 25 - DNA, 20 bp, CNAG_04093 5 flanking region primer 1
tccaggcgtattcatcccag

SEQ ID NO: 26 - DNA, 38 bp, CNAG_04093 5 flanking region primer 2
ctggccgtcgttttacaaggattgtgacctcaggctcg

SEQ ID NO: 27 - DNA, 36 bp, CNAG_04093 3 flanking region primer 1
gtcatagctgtttcctgatgtttctcctccagagcc

SEQ ID NO: 28 - DNA, 19 bp, CNAG_04093 3 flanking region primer 2
gcaagaaccaaatgacagc

SEQ ID NO: 29 - DNA, 24 bp, CNAG_04093 diagnostic screening primer, pairing with B79
atcattcctctgacaagtcgggcg

SEQ ID NO: 30 - DNA, 19 bp, CNAG_04093 Southern blot probe primer
atgtgtcctggatggcttg

SEQ ID NO: 31 - DNA, 20 bp, NAT#5 STM primer
tgctagagggcgggagagtt

SEQ ID NO: 32 - DNA, 24 bp, STM common primer
gcatgccctgcccctaagaattcg

SEQ ID NO: 33 - DNA, 18 bp, CNAG_04518 5 flanking region primer 1
tgtcctttcttgtgaccg

SEQ ID NO: 34 - DNA, 39 bp, CNAG_04518 5 flanking region primer 2
tcactggccgtcgttttaccagtaacgaagaacgcaatc

SEQ ID NO: 35 - DNA, 40 bp, CNAG_04518 3 flanking region primer 1
catggtcatagctgtttcctgcacaagccacgattattgc

SEQ ID NO: 36 - DNA, 20 bp, CNAG_04518 3 flanking region primer 2
tgtatctgtgtgtggactgc

SEQ ID NO: 37 - DNA, 18 bp, CNAG_04518 diagnostic screening primer, pairing with B79
acacaaagggaggaatgc

SEQ ID NO: 38 - DNA, 19 bp, CNAG_04518 Southern blot probe primer
catacactgtgccacgaac

SEQ ID NO: 39 - DNA, 20 bp, NAT#6 STM primer
atagctaccacacgatagct

SEQ ID NO: 40 - DNA, 24 bp, STM common primer
gcatgccctgcccctaagaattcg

SEQ ID NO: 41 - DNA, 20 bp, CNAG_01858 5 flanking region primer 1
tcttcaggaacataggatgg

SEQ ID NO: 42 - DNA, 38 bp, CNAG_01858 5 flanking region primer 2
tcactggccgtcgttttacgagattgttgggaggattg

SEQ ID NO: 43 - DNA, 39 bp, CNAG_01858 3 flanking region primer 1
catggtcatagctgtttcctggggcgaataaggtttctg

SEQ ID NO: 44 - DNA, 18 bp, CNAG_01858 3 flanking region primer 2
tgttttcgctcatccgtc

SEQ ID NO: 45 - DNA, 19 bp, CNAG_01858 diagnostic screening primer, pairing with B79
aacacagcggaatgacctc

SEQ ID NO: 46 - DNA, 18 bp, CNAG_01858 Southern blot probe primer
cacttggttcattgctgg

SEQ ID NO: 47 - DNA, 20 bp, NAT#43 STM primer
ccagctaccaatcacgctac

SEQ ID NO: 48 - DNA, 24 bp, STM common primer
gcatgccctgcccctaagaattcg

SEQ ID NO: 49 - DNA, 22 bp, CNAG_02305 5 flanking region primer 1
ccagaaggatgtgatactgagg

SEQ ID NO: 50 - DNA, 36 bp, CNAG_02305 5 flanking region primer 2
ctggccgtcgttttacgaaatcgttctgaaactgcg

SEQ ID NO: 51 - DNA, 39 bp, CNAG_02305 3 flanking region primer 1
gtcatagctgtttcctgatcgttcacaggctcaaggctg

SEQ ID NO: 52 - DNA, 22 bp, CNAG_02305 3 flanking region primer 2
gaggtcattagagggtatttgc

SEQ ID NO: 53 - DNA, 19 bp, CNAG_02305 diagnostic screening primer, pairing with B79
gcgtggcgaatacatacag

SEQ ID NO: 54 - DNA, 19 bp, CNAG_02305 Southern blot probe primer
aggtgctacaaagactcgg

SEQ ID NO: 55 - DNA, 24 bp, NAT#58 STM primer
cgcaaaatcactagccctatagcg

SEQ ID NO: 56 - DNA, 24 bp, STM common primer
gcatgccctgcccctaagaattcg

SEQ ID NO: 57 - DNA, 19 bp, CNAG_06156 5 flanking region primer 1
aagatagcacctccgacag

SEQ ID NO: 58 - DNA, 41 bp, CNAG_06156 5 flanking region primer 2
gctcactggccgtcgttttacgctgttgcgaaagataaagg

SEQ ID NO: 59 - DNA, 41 bp, CNAG_06156 3 flanking region primer 1
catggtcatagctgtttcctgccaggaatgaactaccaagg

SEQ ID NO: 60 - DNA, 19 bp, CNAG_06156 3 flanking region primer 2
ttgaagcaggactctccac

SEQ ID NO: 61 - DNA, 19 bp, CNAG_06156 diagnostic screening primer, pairing with B79
tgcttgtcgtttggttagg

SEQ ID NO: 62 - DNA, 19 bp, CNAG_06156 Southern blot probe primer
ggtgaaaatgacggtccag

SEQ ID NO: 63 - DNA, 24 bp, NAT#119 STM primer
ctccccacataaagagagctaaac

SEQ ID NO: 64 - DNA, 24 bp, STM common primer
gcatgccctgcccctaagaattcg

SEQ ID NO: 65 - DNA, 21 bp, CNAG_06188 5 flanking region primer 1
ctcttgtcttctgcctattcc

SEQ ID NO: 66 - DNA, 35 bp, CNAG_06188 5 flanking region primer 2
ctggccgtcgttttacggacatagtgaaactgggg

SEQ ID NO: 67 - DNA, 38 bp, CNAG_06188 3 flanking region primer 1
gtcatagctgtttcctgtcatcctccgactctaaactg

SEQ ID NO: 68 - DNA, 20 bp, CNAG_06188 3 flanking region primer 2
gttttcctacttttgtgggc

SEQ ID NO: 69 - DNA, 20 bp, CNAG_06188 diagnostic screening primer, pairing with B79
agaagacgactgtggtaggc

SEQ ID NO: 70 - DNA, 20 bp, CNAG_06188 Southern blot probe primer
gagtcagcagcagaagattc

SEQ ID NO: 71 - DNA, 24 bp, NAT#122 STM primer
acagctccaaacctcgctaaacag

SEQ ID NO: 72 - DNA, 24 bp, STM common primer
gcatgccctgcccctaagaattcg

SEQ ID NO: 73 - DNA, 19 bp, CNAG_05785 5 flanking region primer 1
catttctacttggttgccg

SEQ ID NO: 74 - DNA, 36 bp, CNAG_05785 5 flanking region primer 2
ctggccgtcgttttacaggagaaagtgatggtcggc

SEQ ID NO: 75 - DNA, 39 bp, CNAG_05785 3 flanking region primer 1
gtcatagctgtttcctgttatcgtgagccttcaagcccc

SEQ ID NO: 76 - DNA, 21 bp, CNAG_05785 3 flanking region primer 2
ccattgtagatgtcggttacg

SEQ ID NO: 77 - DNA, 22 bp, CNAG_05785 diagnostic screening primer, pairing with B79
ttgcggtctttgtcccttgtgg

SEQ ID NO: 78 - DNA, 24 bp, CNAG_05785 Southern blot probe primer
ttctccacttgctcgcctatcctc

SEQ ID NO: 79 - DNA, 24 bp, NAT#125 STM primer
cgctacagccagcgcgcgcaagcg

SEQ ID NO: 80 - DNA, 24 bp, STM common primer
gcatgccctgcccctaagaattcg

SEQ ID NO: 81 - DNA, 20 bp, CNAG_05019 5 flanking region primer 1
aaccaccacaatgtcttcag

SEQ ID NO: 82 - DNA, 40 bp, CNAG_05019 5 flanking region primer 2
gctcactggccgtcgttttacagacccttgtttggttctg

SEQ ID NO: 83 - DNA, 41 bp, CNAG_05019 3 flanking region primer 1
catggtcatagctgtttcctgagtggagagggagagcaatg

SEQ ID NO: 84 - DNA, 18 bp, CNAG_05019 3 flanking region primer 2
tttacgaagagcagcgac

SEQ ID NO: 85 - DNA, 18 bp, CNAG_05019 diagnostic screening primer, pairing with B79
agatagcaacggctttgg

SEQ ID NO: 86 - DNA, 20 bp, CNAG_05019 Southern blot probe primer
cgcaaaagggaagatggata

SEQ ID NO: 87 - DNA, 20 bp, NAT#150 STM primer
acatacacccccatcccccc

SEQ ID NO: 88 - DNA, 24 bp, STM common primer
gcatgccctgcccctaagaattcg

SEQ ID NO: 89 - DNA, 18 bp, CNAG_02877 5 flanking region primer 1
gtttaccatttcaccgcc

SEQ ID NO: 90 - DNA, 39 bp, CNAG_02877 5 flanking region primer 2
tcactggccgtcgttttactgatgaggatacattcggag

SEQ ID NO: 91 - DNA, 41 bp, CNAG_02877 3 flanking region primer 1
catggtcatagctgtttcctgggcttcaacaatcaccattc

SEQ ID NO: 92 - DNA, 18 bp, CNAG_02877 3 flanking region primer 2
acgaaaagcggatagcag

SEQ ID NO: 93 - DNA, 20 bp, CNAG_02877 diagnostic screening primer, pairing with B79
agccttattatgaccaaccc

SEQ ID NO: 94 - DNA, 20 bp, CNAG_02877 Southern blot probe primer
caagttcctttgcctacacc

SEQ ID NO: 95 - DNA, 21 bp, NAT#159 STM primer
acgcaccagacacacaaccag

SEQ ID NO: 96 - DNA, 24 bp, STM common primer
gcatgccctgcccctaagaattcg

SEQ ID NO: 97 - DNA, 20 bp, CNAG_00039 5 flanking region primer 1
tcactctttcggggcatcag

SEQ ID NO: 98 - DNA, 38 bp, CNAG_00039 5 flanking region primer 2
ctggccgtcgttttacctaactggggatgaaatgtctg

SEQ ID NO: 99 - DNA, 39 bp, CNAG_00039 3 flanking region primer 1
gtcatagctgtttcctgggggaagagcagaaagagtaac

SEQ ID NO: 100 - DNA, 22 bp, CNAG_00039 3 flanking region primer 2
gcaatcgtaaacaacacccttg

SEQ ID NO: 101 - DNA, 20 bp, CNAG_00039 diagnostic screening primer, pairing with B79
cgtctgtcgtttatcggttg

SEQ ID NO: 102 - DNA, 19 bp, CNAG_00039 Southern blot probe primer
accctgtaacatttgtccg

SEQ ID NO: 103 - DNA, 19 bp, CNAG_00039 Southern blot probe primer
acttacccttcacgccaag

SEQ ID NO: 104 - DNA, 20 bp, NAT#177 STM primer
caccaactccccatctccat

SEQ ID NO: 105 - DNA, 24 bp, STM common primer
gcatgccctgcccctaagaattcg

SEQ ID NO: 106 - DNA, 20 bp, CNAG_00039 5 flanking region primer 1
agacattgggcttgacggtg

SEQ ID NO: 107 - DNA, 39 bp, CNAG_00039 5 flanking region primer 2
tcactggccgtcgttttacacgagttggagaggggttac

SEQ ID NO: 108 - DNA, 39 bp, CNAG_00039 3 flanking region primer 1
catggtcatagctgtttcctgtagaaaggaatcggggac

SEQ ID NO: 109 - DNA, 20 bp, CNAG_00039 3 flanking region primer 2
ggagaacgaaaacaaagtgc

SEQ ID NO: 110 - DNA, 19 bp, CNAG_00039 diagnostic screening primer, pairing with B79
ggttcttgtttatgccctg

SEQ ID NO: 111 - DNA, 20 bp, CNAG_00039 Southern blot probe primer
aacgagggtagattgcgtcg

SEQ ID NO: 112 - DNA, 20 bp, NAT#177 STM primer
caccaactccccatctccat

SEQ ID NO: 113 - DNA, 24 bp, STM common primer
gcatgccctgcccctaagaattcg

SEQ ID NO: 114 - DNA, 19 bp, CNAG_01014 5 flanking region primer 1
tatcgccgacatctctcag

SEQ ID NO: 115 - DNA, 38 bp, CNAG_01014 5 flanking region primer 2
tcactggccgtcgttttactttaggacggaggggattg

SEQ ID NO: 116 - DNA, 39 bp, CNAG_01014 3 flanking region primer 1
catggtcatagctgtttcctggagccgaatcaggaaatc

SEQ ID NO: 117 - DNA, 19 bp, CNAG_01014 3 flanking region primer 2
cgcaggcttttctactctc

SEQ ID NO: 118 - DNA, 30 bp, CNAG_01014 diagnostic screening primer, pairing with B79
cgcgcggccgcgaaaacctccacagagcag

SEQ ID NO: 119 - DNA, 19 bp, CNAG_01014 Southern blot probe primer
ttgcttgctgtctcgtaac

SEQ ID NO: 120 - DNA, 18 bp, CNAG_01014 Southern blot probe primer
gatttcctgattcggctc

SEQ ID NO: 121 - DNA, 20 bp, CTAGAGCCCGCCACAACGCT
ctagagcccgccacaacgct

SEQ ID NO: 122 - DNA, 24 bp, STM common primer
gcatgccctgcccctaagaattcg

SEQ ID NO: 123 - DNA, 21 bp, CNAG_06762 5 flanking region primer 1
tgggtgagagaaagatgtcag

SEQ ID NO: 124 - DNA, 39 bp, CNAG_06762 5 flanking region primer 2
tcactggccgtcgttttactgtgagtggttgtgctgtgg

SEQ ID NO: 125 - DNA, 41 bp, CNAG_06762 3 flanking region primer 1
catggtcatagctgtttcctgggctcataggtgttgtaacg

SEQ ID NO: 126 - DNA, 20 bp, CNAG_06762 3 flanking region primer 2
agtattcggtggtgacaaag

SEQ ID NO: 127 - DNA, 21 bp, CNAG_06762 diagnostic screening primer, pairing with B79
tgggtgagagaaagatgtcag

SEQ ID NO: 128 - DNA, 19 bp, CNAG_06762 Southern blot probe primer
tgttccaccccttgctaac

SEQ ID NO: 129 - DNA, 20 bp, NAT#218 STM primer
ctccacatccatcgctccaa

SEQ ID NO: 130 - DNA, 24 bp, STM common primer
gcatgccctgcccctaagaattcg

SEQ ID NO: 131 - DNA, 18 bp, CNAG_04630 5 flanking region primer 1
atggaaggactttgacgg

SEQ ID NO: 132 - DNA, 40 bp, CNAG_04630 5 flanking region primer 2
tcactggccgtcgttttactgactcacacttgattctccc

SEQ ID NO: 133 - DNA, 40 bp, CNAG_04630 3 flanking region primer 1
gatggtcatagctgtttcctgctcattttccctttcgtcg

SEQ ID NO: 134 - DNA, 18 bp, CNAG_04630 3 flanking region primer 2
taaaggaatgcggctgag

SEQ ID NO: 135 - DNA, 19 bp, CNAG_04630 diagnostic screening primer, pairing with B79
ccaacagcaacttcgtttc

SEQ ID NO: 136 - DNA, 21 bp, CNAG_04630 Southern blot probe primer
tctcttctccttggaactgag

SEQ ID NO: 137 - DNA, 20 bp, NAT#218 STM primer
ctccacatccatcgctccaa

SEQ ID NO: 138 - DNA, 24 bp, STM common primer
gcatgccctgcccctaagaattcg

SEQ ID NO: 139 - DNA, 19 bp, CNAG_03401 5 flanking region primer 1
ttcctcgtccaagtaaacc

SEQ ID NO: 140 - DNA, 41 bp, CNAG_03401 5 flanking region primer 2
gctcactggccgtcgttttacaatctcgcaaaccgcacacg

SEQ ID NO: 141 - DNA, 43 bp, CNAG_03401 3 flanking region primer 1
catggtcatagctgtttcctgagcgcgaacagggaaatacacc

SEQ ID NO: 142 - DNA, 18 bp, CNAG_03401 3 flanking region primer 2
tcgtgtaggaatgggtag

SEQ ID NO: 143 - DNA, 20 bp, CNAG_03401 diagnostic screening primer, pairing with B79
tggtctccccgacgatttac

SEQ ID NO: 144 - DNA, 19 bp, CNAG_03401 Southern blot probe primer
tatggtcaggaggaagcag

SEQ ID NO: 145 - DNA, 20 bp, NAT#220 STM primer
cagatctcgaacgataccca

SEQ ID NO: 146 - DNA, 24 bp, STM common primer
gcatgccctgcccctaagaattcg

SEQ ID NO: 147 - DNA, 22 bp, CNAG_04594 5 flanking region primer 1
tggcatcgtgctgttacaagtc

SEQ ID NO: 148 - DNA, 45 bp, CNAG_04594 5 flanking region primer 2
gctcactggccgtcgttttacatttgcggatggacctgccttagg

SEQ ID NO: 149 - DNA, 41 bp, CNAG_04594 3 flanking region primer 1
catggtcatagctgtttcctgatcaggattcaggacacgac

SEQ ID NO: 150 - DNA, 18 bp, CNAG_04594 3 flanking region primer 2
tttggttctctctcccac

SEQ ID NO: 151 - DNA, 19 bp, CNAG_04594 diagnostic screening primer, pairing with B79
attgcttgagaccagcgtc

SEQ ID NO: 152 - DNA, 18 bp, CNAG_04594 Southern blot probe primer
acggttgctttgctatgc

SEQ ID NO: 153 - DNA, 20 bp, NAT#220 STM primer
cagatctcgaacgataccca

SEQ ID NO: 154 - DNA, 24 bp, STM common primer
gcatgccctgcccctaagaattcg

SEQ ID NO: 155 - DNA, 19 bp, CNAG_07901 5 flanking region primer 1
actcaccttcccgctttag

SEQ ID NO: 156 - DNA, 34 bp, CNAG_07901 5 flanking region primer 2
ctggccgtcgttttacgtttgagttgaggttgcg

SEQ ID NO: 157 - DNA, 36 bp, CNAG_07901 3 flanking region primer 1
gtcatagctgtttcctgagaatgttgatggtagcgg

SEQ ID NO: 158 - DNA, 19 bp, CNAG_07901 3 flanking region primer 2
tccaccgaagaaactgaag

SEQ ID NO: 159 - DNA, 18 bp, CNAG_07901 diagnostic screening primer, pairing with B79
gggatttggatacgcttg

SEQ ID NO: 160 - DNA, 18 bp, CNAG_07901 Southern blot probe primer
ttgcggtgggaaagtatc

SEQ ID NO: 161 - DNA, 20 bp, NAT#225 STM primer
ccatagaactagctaaagca

SEQ ID NO: 162 - DNA, 24 bp, STM common primer
gcatgccctgcccctaagaattcg

SEQ ID NO: 163 - DNA, 19 bp, CNAG_04588 5 flanking region primer 1
aaaagaggtccgatgagtg

SEQ ID NO: 164 - DNA, 40 bp, CNAG_04588 5 flanking region primer 2
gctcactggccgtcgttttacgtgaatgataaaggcgacc

SEQ ID NO: 165 - DNA, 39 bp, CNAG_04588 3 flanking region primer 1
catggtcatagctgtttcctgtgctgtttcactatccgc

SEQ ID NO: 166 - DNA, 19 bp, CNAG_04588 3 flanking region primer 2
cgaaagcgactggagtaac

SEQ ID NO: 167 - DNA, 20 bp, CNAG_04588 diagnostic screening primer, pairing with B79
gaagatgctgaagcgtattc

SEQ ID NO: 168 - DNA, 18 bp, CNAG_04588 Southern blot probe primer
acacttatccgccattcc

SEQ ID NO: 169 - DNA, 20 bp, NAT#225 STM primer
ccatagaactagctaaagca

SEQ ID NO: 170 - DNA, 24 bp, STM common primer
gcatgccctgcccctaagaattcg

SEQ ID NO: 171 - DNA, 18 bp, CNAG_03998 5 flanking region primer 1
gccattgtgaaagcatag

SEQ ID NO: 172 - DNA, 43 bp, CNAG_03998 5 flanking region primer 2
gctcactggccgtcgttttacacctgtctatctcactgtccag

SEQ ID NO: 173 - DNA, 39 bp, CNAG_03998 3 flanking region primer 1
catggtcatagctgtttcctgtgttcagcagcaaaaggc

SEQ ID NO: 174 - DNA, 18 bp, CNAG_03998 3 flanking region primer 2
gcggagagaaggattatc

SEQ ID NO: 175 - DNA, 20 bp, CNAG_03998 diagnostic screening primer, pairing with B79
gctgacaacttggaatcatc

SEQ ID NO: 176 - DNA, 20 bp, CNAG_03998 Southern blot probe primer
gggcttctcttcttcttcac

SEQ ID NO: 177 - DNA, 20 bp, NAT#234 STM primer
ccagccagcactccgatata

SEQ ID NO: 178 - DNA, 24 bp, STM common primer
gcatgccctgcccctaagaattcg

SEQ ID NO: 179 - DNA, 20 bp, CNAG_04804 5 flanking region primer 1
taggtagttcctgctcgtgg

SEQ ID NO: 180 - DNA, 40 bp, CNAG_04804 5 flanking region primer 2
tcactggccgtcgttttaccatcttgtcctgtaatgaggc

SEQ ID NO: 181 - DNA, 39 bp, CNAG_04804 3 flanking region primer 1
catggtcatagctgtttcctggattggagggcgatttag

SEQ ID NO: 182 - DNA, 20 bp, CNAG_04804 3 flanking region primer 2
caacaaggtccaagaaactg

SEQ ID NO: 183 - DNA, 21 bp, CNAG_04804 diagnostic screening primer, pairing with B79
agaggactgagacttttgtcg

SEQ ID NO: 184 - DNA, 19 bp, CNAG_04804 Southern blot probe primer
cgaaggggaactggttatc

SEQ ID NO: 185 - DNA, 20 bp, NAT#240 STM primer
ggtgttggatcggggtggat

SEQ ID NO: 186 - DNA, 24 bp, STM common primer
gcatgccctgcccctaagaattcg

SEQ ID NO: 187 - DNA, 20 bp, CNAG_06134 5 flanking region primer 1
gtttgaggctggtaaaaagg

SEQ ID NO: 188 - DNA, 39 bp, CNAG_06134 5 flanking region primer 2
gctcactggccgtcgttttacatggggaatgaaagcgtg

SEQ ID NO: 189 - DNA, 41 bp, CNAG_06134 3 flanking region primer 1
catggtcatagctgtttcctgaaggggcgagagtagttcag

SEQ ID NO: 190 - DNA, 21 bp, CNAG_06134 3 flanking region primer 2
gactgtaaaggagggcataag

SEQ ID NO: 191 - DNA, 19 bp, CNAG_06134 diagnostic screening primer, pairing with B79
aactcttctcagccttcgg

SEQ ID NO: 192 - DNA, 19 bp, CNAG_06134 Southern blot probe primer
cgttctccgtcttgatagc

SEQ ID NO: 193 - DNA, 21 bp, NAT#295 STM primer
acacctacatcaaaccctccc

SEQ ID NO: 194 - DNA, 24 bp, STM common primer
gcatgccctgcccctaagaattcg

SEQ ID NO: 195 - DNA, 19 bp, CNAG_04798 5 flanking region primer 1
caatgattaggcttgcgtc

SEQ ID NO: 196 - DNA, 38 bp, CNAG_04798 5 flanking region primer 2
tcactggccgtcgttttactgttgttgggcagtggtag

SEQ ID NO: 197 - DNA, 39 bp, CNAG_04798 3 flanking region primer 1
catggtcatagctgtttcctgtttagggaagaggaagcg

SEQ ID NO: 198 - DNA, 18 bp, CNAG_04798 3 flanking region primer 2
tgtcatccagcagattgg

SEQ ID NO: 199 - DNA, 19 bp, CNAG_04798 diagnostic screening primer, pairing with B79
tgaatgactgatggacccc

SEQ ID NO: 200 - DNA, 18 bp, CNAG_04798 Southern blot probe primer
tcggttctcgttttggag

SEQ ID NO: 201 - DNA, 20 bp, CNAG_04864 5 flanking region primer 1
tcatttcttcgtcctctgag

SEQ ID NO: 202 - DNA, 36 bp, CNAG_04864 5 flanking region primer 2
ctggccgtcgttttacgctccccataatcagactcc

SEQ ID NO: 203 - DNA, 36 bp, CNAG_04864 3 flanking region primer 1
gtcatagctgtttcctgacgaatggagtttctggag

SEQ ID NO: 204 - DNA, 20 bp, CNAG_04864 3 flanking region primer 2
gcgttctccatagttgtagc

SEQ ID NO: 205 - DNA, 20 bp, CNAG_04864 diagnostic screening primer, pairing with B79
atgtagataaagcacgcacc

SEQ ID NO: 206 - DNA, 20 bp, CNAG_04864 Southern blot probe primer
cgagttattgtaggttgggc

SEQ ID NO: 207 - DNA, 20 bp, CNAG_01973 5 flanking region primer 1
gcttgaggttgaaacaggtc

SEQ ID NO: 208 - DNA, 41 bp, CNAG_01973 5 flanking region primer 2
tcactggccgtcgttttaccagatgtgtgtaagagggtcag

SEQ ID NO: 209 - DNA, 39 bp, CNAG_01973 3 flanking region primer 1
catggtcatagctgtttcctgtaccgagaacgatttggc

SEQ ID NO: 210 - DNA, 20 bp, CNAG_01973 3 flanking region primer 2
tcccataagaccacacactg

SEQ ID NO: 211 - DNA, 19 bp, CNAG_01973 diagnostic screening primer, pairing with B79
tgatgctgaatagacgggg

SEQ ID NO: 212 - DNA, 19 bp, CNAG_01973 Southern blot probe primer
agccttgacgacatacctg

SEQ ID NO: 213 - DNA, 20 bp, NAT#6 STM primer
atagctaccacacgatagct

SEQ ID NO: 214 - DNA, 24 bp, STM common primer
gcatgccctgcccctaagaattcg

SEQ ID NO: 215 - DNA, 19 bp, CNAG_03914 5 flanking region primer 1
gatgtcgttgttccagagc

SEQ ID NO: 216 - DNA, 35 bp, CNAG_03914 5 flanking region primer 2
ctggccgtcgttttactttggatgtaagaggtcgg

SEQ ID NO: 217 - DNA, 37 bp, CNAG_03914 3 flanking region primer 1
gtcatagctgtttcctgcgagtatccttaccgtgtcg

SEQ ID NO: 218 - DNA, 19 bp, CNAG_03914 3 flanking region primer 2
acactcctgcccaagaaac

SEQ ID NO: 219 - DNA, 19 bp, CNAG_03914 diagnostic screening primer, pairing with B79
actccactccatccaaagc

SEQ ID NO: 220 - DNA, 20 bp, CNAG_03914 Southern blot probe primer
ataagaggtccttttgctcc

SEQ ID NO: 221 - DNA, 20 bp, NAT#43 STM primer
ccagctaccaatcacgctac

SEQ ID NO: 222 - DNA, 24 bp, STM common primer
gcatgccctgcccctaagaattcg

SEQ ID NO: 223 - DNA, 19 bp, CNAG_00828 5 flanking region primer 1
accagtggcaaggttagag

SEQ ID NO: 224 - DNA, 39 bp, CNAG_00828 5 flanking region primer 2
tcactggccgtcgttttactggcagaagcacaagattag

SEQ ID NO: 225 - DNA, 40 bp, CNAG_00828 3 flanking region primer 1
catggtcatagctgtttcctggccatttctcgtagcgaac

SEQ ID NO: 226 - DNA, 19 bp, CNAG_00828 3 flanking region primer 2
actgcttatccccacatcg

SEQ ID NO: 227 - DNA, 20 bp, CNAG_00828 diagnostic screening primer, pairing with B79
tgtgaagtgtgatgatgtcc

SEQ ID NO: 228 - DNA, 19 bp, CNAG_00828 Southern blot probe primer
ggttgccactgataaaagc

SEQ ID NO: 229 - DNA, 24 bp, NAT#58 STM primer
cgcaaaatcactagccctatagcg

SEQ ID NO: 230 - DNA, 24 bp, STM common primer
gcatgccctgcccctaagaattcg

SEQ ID NO: 231 - DNA, 19 bp, CNAG_00871 5 flanking region primer 1
atagcgggcaagtgtctac

SEQ ID NO: 232 - DNA, 38 bp, CNAG_00871 5 flanking region primer 2
tcactggccgtcgttttacccaacctttcattccagtc

SEQ ID NO: 233 - DNA, 42 bp, CNAG_00871 3 flanking region primer 1
catggtcatagctgtttcctgggatacaaatctcaacccctg

SEQ ID NO: 234 - DNA, 19 bp, CNAG_00871 3 flanking region primer 2
ggttttcacttcaagagcg

SEQ ID NO: 235 - DNA, 18 bp, CNAG_00871 diagnostic screening primer, pairing with B79
tccaatagcaccacaacc

SEQ ID NO: 236 - DNA, 19 bp, CNAG_00871 Southern blot probe primer
aacatccctttactcggcg

SEQ ID NO: 237 - DNA, 24 bp, NAT#102 STM primer
ccatagcgatatctaccccaatct

SEQ ID NO: 238 - DNA, 24 bp, STM common primer
gcatgccctgcccctaagaattcg

SEQ ID NO: 239 - DNA, 19 bp, CNAG_07464 5 flanking region primer 1
ggcatcaggatagaaacgc

SEQ ID NO: 240 - DNA, 41 bp, CNAG_07464 5 flanking region primer 2
gctcactggccgtcgttttacggggtgagatttgaaggtag

SEQ ID NO: 241 - DNA, 40 bp, CNAG_07464 3 flanking region primer 1
catggtcatagctgtttcctggatgtgacttggtcttggg

SEQ ID NO: 242 - DNA, 20 bp, CNAG_07464 3 flanking region primer 2
tggtccagtctcctcattac

SEQ ID NO: 243 - DNA, 18 bp, CNAG_07464 diagnostic screening primer, pairing with B79
tcttccatctcagcatcg

SEQ ID NO: 244 - DNA, 24 bp, CNAG_07464 Southern blot probe primer
ccatagcgatatctaccccaatct

SEQ ID NO: 245 - DNA, 20 bp, NAT#150 STM primer
acatacacccccatcccccc

SEQ ID NO: 246 - DNA, 24 bp, STM common primer
gcatgccctgcccctaagaattcg

SEQ ID NO: 247 - DNA, 23 bp, CNAG_00460 5 flanking region primer 1
cgtgggagagtgagtaaagtatg

SEQ ID NO: 248 - DNA, 42 bp, CNAG_00460 5 flanking region primer 2
gctcactggccgtcgttttaccgggtaagagtggatgtatgg

SEQ ID NO: 249 - DNA, 39 bp, CNAG_00460 3 flanking region primer 1
catggtcatagctgtttcctgaagggcaccgttcattag

SEQ ID NO: 250 - DNA, 19 bp, CNAG_00460 3 flanking region primer 2
ttcttaggatgcgggactc

SEQ ID NO: 251 - DNA, 18 bp, CNAG_00460 diagnostic screening primer, pairing with B79
tgcgttgacaaagtcgtg

SEQ ID NO: 252 - DNA, 22 bp, CNAG_00460 Southern blot probe primer
tagactccagtaaggtccaatc

SEQ ID NO: 253 - DNA, 24 bp, NAT#213 STM primer
ctggggattttgatgtgtctatgt

SEQ ID NO: 254 - DNA, 24 bp, STM common primer
gcatgccctgcccctaagaattcg

SEQ ID NO: 255 - DNA, 18 bp, CNAG_01431 5 flanking region primer 1
tccatttgggggtttcag

SEQ ID NO: 256 - DNA, 39 bp, CNAG_01431 5 flanking region primer 2
tcactggccgtcgttttactgtcttcgttcttgccctcc

SEQ ID NO: 257 - DNA, 42 bp, CNAG_01431 3 flanking region primer 1
catggtcatagctgtttcctgcgttgacagaagaggacaagg

SEQ ID NO: 258 - DNA, 20 bp, CNAG_01431 3 flanking region primer 2
tgacagatgatgagcagagg

SEQ ID NO: 259 - DNA, 19 bp, CNAG_01431 diagnostic screening primer, pairing with B79
attccagagcctcacttgc

SEQ ID NO: 260 - DNA, 21 bp, CNAG_01431 Southern blot probe primer
cctgcttgtcactacactgag

SEQ ID NO: 261 - DNA, 24 bp, NAT#213 STM primer
ctggggattttgatgtgtctatgt

SEQ ID NO: 262 - DNA, 24 bp, STM common primer
gcatgccctgcccctaagaattcg

SEQ ID NO: 263 - DNA, 21 bp, CNAG_03894 5 flanking region primer 1
catctatctcaacggggtatc

SEQ ID NO: 264 - DNA, 39 bp, CNAG_03894 5 flanking region primer 2
gctcactggccgtcgttttactttttcgggagaacgcag

SEQ ID NO: 265 - DNA, 40 bp, CNAG_03894 3 flanking region primer 1
catggtcatagctgtttcctgaggaccaagaatgctgagg

SEQ ID NO: 266 - DNA, 22 bp, CNAG_03894 3 flanking region primer 2
ttctcccttgtcgccgataagc

SEQ ID NO: 267 - DNA, 20 bp, CNAG_03894 diagnostic screening primer, pairing with B79
tcttatcgctcaccacatcc

SEQ ID NO: 268 - DNA, 19 bp, CNAG_03894 Southern blot probe primer
ggaacattgggaaaaggtg

SEQ ID NO: 269 - DNA, 20 bp, NAT#220 STM primer
cagatctcgaacgataccca

SEQ ID NO: 270 - DNA, 24 bp, STM common primer
gcatgccctgcccctaagaattcg

SEQ ID NO: 271 - DNA, 18 bp, CNAG_06483 5 flanking region primer 1
tggagcagatggagtttg

SEQ ID NO: 272 - DNA, 35 bp, CNAG_06483 5 flanking region primer 2
ctggccgtcgttttacgcttctccctatttccagc

SEQ ID NO: 273 - DNA, 36 bp, CNAG_06483 3 flanking region primer 1
gtcatagctgtttcctgaatggagcccagagaacag

SEQ ID NO: 274 - DNA, 19 bp, CNAG_06483 3 flanking region primer 2
tctcgctgagggaaaactc

SEQ ID NO: 275 - DNA, 18 bp, CNAG_06483 diagnostic screening primer, pairing with B79
ccctttctctgcgttttg

SEQ ID NO: 276 - DNA, 18 bp, CNAG_06483 Southern blot probe primer
caatgaagaactggtgcg

SEQ ID NO: 277 - DNA, 20 bp, NAT#227 STM primer
tcgtggtttagagggagcgc

SEQ ID NO: 278 - DNA, 24 bp, STM common primer
gcatgccctgcccctaagaattcg

SEQ ID NO: 279 - DNA, 18 bp, CNAG_00896 5 flanking region primer 1
aaagggtcacgatggaac

SEQ ID NO: 280 - DNA, 35 bp, CNAG_00896 5 flanking region primer 2
ctggccgtcgttttacgcgattctttactcctggc

SEQ ID NO: 281 - DNA, 36 bp, CNAG_00896 3 flanking region primer 1
gtcatagctgtttcctgttctgagacctccgtaacc

SEQ ID NO: 282 - DNA, 19 bp, CNAG_00896 3 flanking region primer 2
ctgtatcgctttagccacc

SEQ ID NO: 283 - DNA, 19 bp, CNAG_00896 diagnostic screening primer, pairing with B79
tacaaggacctcacgaacg

SEQ ID NO: 284 - DNA, 20 bp, CNAG_00896 Southern blot probe primer
acgagcagagggacagatag

SEQ ID NO: 285 - DNA, 20 bp, NAT#231 STM primer
gagagatcccaacatcacgc

SEQ ID NO: 286 - DNA, 24 bp, STM common primer
gcatgccctgcccctaagaattcg

SEQ ID NO: 287 - DNA, 18 bp, CNAG_01977 5 flanking region primer 1
tgggaaaacgaagcactc

SEQ ID NO: 288 - DNA, 35 bp, CNAG_01977 5 flanking region primer 2
ctggccgtcgttttactaggaggtcactttcgctc

SEQ ID NO: 289 - DNA, 36 bp, CNAG_01977 3 flanking region primer 1
gtcatagctgtttcctgcggcaaagaacaaggtatg

SEQ ID NO: 290 - DNA, 20 bp, CNAG_01977 3 flanking region primer 2
tgatgggcttgaacgaacgc

SEQ ID NO: 291 - DNA, 19 bp, CNAG_01977 diagnostic screening primer, pairing with B79
tgtcggcacacatctactg

SEQ ID NO: 292 - DNA, 22 bp, CNAG_01977 Southern blot probe primer
gtctcagcctcttgttacagat

SEQ ID NO: 293 - DNA, 20 bp, NAT#231 STM primer
gagagatcccaacatcacgc

SEQ ID NO: 294 - DNA, 24 bp, STM common primer
gcatgccctgcccctaagaattcg

SEQ ID NO: 295 - DNA, 19 bp, CNAG_01069 5 flanking region primer 1
cttttatctatggcgagcg

SEQ ID NO: 296 - DNA, 39 bp, CNAG_01069 5 flanking region primer 2
gctcactggccgtcgttttactatcgcactgctggaatc

SEQ ID NO: 297 - DNA, 40 bp, CNAG_01069 3 flanking region primer 1
catggtcatagctgtttcctgctactttccctcacatccg

SEQ ID NO: 298 - DNA, 19 bp, CNAG_01069 3 flanking region primer 2
tggagggtagatgcgttac

SEQ ID NO: 299 - DNA, 20 bp, CNAG_01069 diagnostic screening primer, pairing with B79
agagaagcggaagagaaaac

SEQ ID NO: 300 - DNA, 20 bp, CNAG_01069 Southern blot probe primer
ccttgcgaaaatgtcttctc

SEQ ID NO: 301 - DNA, 21 bp, NAT#292 STM primer
atttcgatgtatatatgtagc

SEQ ID NO: 302 - DNA, 24 bp, STM common primer
gcatgccctgcccctaagaattcg

SEQ ID NO: 303 - DNA, 19 bp, CNAG_06276 5 flanking region primer 1
tcaagtctacgcagtcgtg

SEQ ID NO: 304 - DNA, 40 bp, CNAG_06276 5 flanking region primer 2
gctcactggccgtcgttttacgcagcaatcaactcactcg

SEQ ID NO: 305 - DNA, 41 bp, CNAG_06276 3 flanking region primer 1
catggtcatagctgtttcctgaggagagtgggagtatggag

SEQ ID NO: 306 - DNA, 18 bp, CNAG_06276 3 flanking region primer 2
acccatcaaaaggcgtag

SEQ ID NO: 307 - DNA, 20 bp, CNAG_06276 diagnostic screening primer, pairing with B79
accatttgtcaactgtcagg

SEQ ID NO: 308 - DNA, 20 bp, CNAG_06276 Southern blot probe primer
tcgctcactgacaagaagac

SEQ ID NO: 309 - DNA, 21 bp, NAT#292 STM primer
atttcgatgtatatatgtagc

SEQ ID NO: 310 - DNA, 24 bp, STM common primer
gcatgccctgcccctaagaattcg

SEQ ID NO: 311 - DNA, 19 bp, CNAG_02476 5 flanking region primer 1
tctgctcaatgaaacgggc

SEQ ID NO: 312 - DNA, 45 bp, CNAG_02476 5 flanking region primer 2
gctcactggccgtcgttttacgcctttgcttcctttgcttcttac

SEQ ID NO: 313 - DNA, 40 bp, CNAG_02476 3 flanking region primer 1
catggtcatagctgtttcctggtgtcttgaatccaatgcc

SEQ ID NO: 314 - DNA, 20 bp, CNAG_02476 3 flanking region primer 2
ctgctccatacaaggcttag

SEQ ID NO: 315 - DNA, 20 bp, CNAG_02476 diagnostic screening primer, pairing with B79
tcgtcagcaattgaaaacct

SEQ ID NO: 316 - DNA, 19 bp, CNAG_02476 Southern blot probe primer
atcaagtcagaccacgagg

SEQ ID NO: 317 - DNA, 20 bp, NAT#219 STM primer
ccctaaaaccctacagcaat

SEQ ID NO: 318 - DNA, 24 bp, STM common primer
gcatgccctgcccctaagaattcg

SEQ ID NO: 319 - DNA, 20 bp, CNAG_01841 5 flanking region primer 1
ccattatcatccgtcaccac

SEQ ID NO: 320 - DNA, 37 bp, CNAG_01841 5 flanking region primer 2
ctggccgtcgttttacgaagagggaagagagggtaac

SEQ ID NO: 321 - DNA, 36 bp, CNAG_01841 3 flanking region primer 1
gtcatagctgtttcctgtgaggctgaggaaacagag

SEQ ID NO: 322 - DNA, 18 bp, CNAG_01841 3 flanking region primer 2
tccttttcccaacctgtc

SEQ ID NO: 323 - DNA, 21 bp, CNAG_01841 diagnostic screening primer, pairing with B79
ttcagtggttggtctctacag

SEQ ID NO: 324 - DNA, 21 bp, CNAG_01841 Southern blot probe primer
tggtaaaggtctatcagtgcc

SEQ ID NO: 325 - DNA, 20 bp, NAT#230 STM primer
atgtaggtagggtgataggt

SEQ ID NO: 326 - DNA, 24 bp, STM common primer
gcatgccctgcccctaagaattcg

SEQ ID NO: 327 - DNA, 19 bp, CNAG_04457 5 flanking region primer 1
cttcaaaatccagagcagg

SEQ ID NO: 328 - DNA, 38 bp, CNAG_04457 5 flanking region primer 2
ctggccgtcgttttacctggtctgatagttcgtattcg

SEQ ID NO: 329 - DNA, 39 bp, CNAG_04457 3 flanking region primer 1
gtcatagctgtttcctgggacttgaacaatggtatggac

SEQ ID NO: 330 - DNA, 19 bp, CNAG_04457 3 flanking region primer 2
tttagagcctacggtggtc

SEQ ID NO: 331 - DNA, 22 bp, CNAG_04457 diagnostic screening primer, pairing with B79
ttgcccgacgagatgctatgac

SEQ ID NO: 332 - DNA, 20 bp, CNAG_04457 Southern blot probe primer
tccgtctccgatgatttgcg

SEQ ID NO: 333 - DNA, 20 bp, NAT#230 STM primer
atgtaggtagggtgataggt

SEQ ID NO: 334 - DNA, 24 bp, STM common primer
gcatgccctgcccctaagaattcg

SEQ ID NO: 335 - DNA, 19 bp, CNAG_06252 5 flanking region primer 1
tctgacaggttcaatcgcc

SEQ ID NO: 336 - DNA, 41 bp, CNAG_06252 5 flanking region primer 2
tcactggccgtcgttttacgcatttctacaccgtgattagc

SEQ ID NO: 337 - DNA, 40 bp, CNAG_06252 3 flanking region primer 1
catggtcatagctgtttcctgggatgtgcggttttgttag

SEQ ID NO: 338 - DNA, 19 bp, CNAG_06252 3 flanking region primer 2
taacgaagttctccccgtg

SEQ ID NO: 339 - DNA, 20 bp, CNAG_06252 diagnostic screening primer, pairing with B79
tgagagggaacgaaggatac

SEQ ID NO: 340 - DNA, 20 bp, CNAG_06252 Southern blot probe primer
cttcgcctgttggaaataag

SEQ ID NO: 341 - DNA, 20 bp, CNAG_06327 5 flanking region primer 1
ggagaagggaaagatgggtg

SEQ ID NO: 342 - DNA, 41 bp, CNAG_06327 5 flanking region primer 2
gctcactggccgtcgttttactgtttccactattgggagag

SEQ ID NO: 343 - DNA, 40 bp, CNAG_06327 3 flanking region primer 1
catggtcatagctgtttcctgaggtgaaggtgtgagattg

SEQ ID NO: 344 - DNA, 18 bp, CNAG_06327 3 flanking region primer 2
caataatgtcctcgccag

SEQ ID NO: 345 - DNA, 19 bp, CNAG_06327 diagnostic screening primer, pairing with B79
gtatgaagggaaggtgctg

SEQ ID NO: 346 - DNA, 18 bp, CNAG_06327 Southern blot probe primer
acgggttacgagaaatgc

SEQ ID NO: 347 - DNA, 19 bp, CNAG_03790 5 flanking region primer 1
tgagggttgttgagggaag

SEQ ID NO: 348 - DNA, 40 bp, CNAG_03790 5 flanking region primer 2
gctcactggccgtcgttttacagcactgtatcgccgaaac

SEQ ID NO: 349 - DNA, 42 bp, CNAG_03790 3 flanking region primer 1
catggtcatagctgtttcctgctcgtagcaatgtagatgtgc

SEQ ID NO: 350 - DNA, 21 bp, CNAG_03790 3 flanking region primer 2
tcagatgaagacgactacgac

SEQ ID NO: 351 - DNA, 19 bp, CNAG_03790 diagnostic screening primer, pairing with B79
cttccacaaagccagattc

SEQ ID NO: 352 - DNA, 18 bp, CNAG_03790 Southern blot probe primer
agattgcgtgaaacccac

SEQ ID NO: 353 - DNA, 19 bp, CNAG_05112 5 flanking region primer 1
atgtgcgaagtccaagagc

SEQ ID NO: 354 - DNA, 40 bp, CNAG_05112 5 flanking region primer 2
gctcactggccgtcgttttacgggtgaagacaacagatgg

SEQ ID NO: 355 - DNA, 41 bp, CNAG_05112 3 flanking region primer 1
catggtcatagctgtttcctgcagaccaactggcgtaatag

SEQ ID NO: 356 - DNA, 19 bp, CNAG_05112 3 flanking region primer 2
acgaccaaatgctcttcgc

SEQ ID NO: 357 - DNA, 19 bp, CNAG_05112 diagnostic screening primer, pairing with B79
tcggatacaggcgatagag

SEQ ID NO: 358 - DNA, 19 bp, CNAG_05112 Southern blot probe primer
tcaacagcagtttcaggtg

SEQ ID NO: 359 - DNA, 24 bp, NAT#122 STM primer
acagctccaaacctcgctaaacag

SEQ ID NO: 360 - DNA, 24 bp, STM common primer
gcatgccctgcccctaagaattcg

SEQ ID NO: 361 - DNA, 19 bp, CNAG_00068 5 flanking region primer 1
tctatcacctctgcgttgc

SEQ ID NO: 362 - DNA, 39 bp, CNAG_00068 5 flanking region primer 2
tcactggccgtcgttttacattcctaccactatcccctg

SEQ ID NO: 363 - DNA, 40 bp, CNAG_00068 3 flanking region primer 1
catggtcatagctgtttcctgcggataagatgcctgagac

SEQ ID NO: 364 - DNA, 22 bp, CNAG_00068 3 flanking region primer 2
ggtatgtttctcggatgtaagg

SEQ ID NO: 365 - DNA, 20 bp, CNAG_00068 diagnostic screening primer, pairing with B79
catcatcaggtatcagcagc

SEQ ID NO: 366 - DNA, 20 bp, CNAG_00068 Southern blot probe primer
cttccaacttcaatgttccc

SEQ ID NO: 367 - DNA, 24 bp, NAT#58 STM primer
cgcaaaatcactagccctatagcg

SEQ ID NO: 368 - DNA, 24 bp, STM common primer
gcatgccctgcccctaagaattcg

SEQ ID NO: 369 - DNA, 19 bp, CNAG_04184 5 flanking region primer 1
tcgttcacataactgccac

SEQ ID NO: 370 - DNA, 38 bp, CNAG_04184 5 flanking region primer 2
tcactggccgtcgttttactcattgtgagcctcgtatg

SEQ ID NO: 371 - DNA, 39 bp, CNAG_04184 3 flanking region primer 1
catggtcatagctgtttcctgaatggtgacggttcaagg

SEQ ID NO: 372 - DNA, 18 bp, CNAG_04184 3 flanking region primer 2
cttttccactgaatccgc

SEQ ID NO: 373 - DNA, 19 bp, CNAG_04184 diagnostic screening primer, pairing with B79
tggtccgatgccgtaaatc

SEQ ID NO: 374 - DNA, 19 bp, CNAG_04184 Southern blot probe primer
caagggaatgactcactcc

SEQ ID NO: 375 - DNA, 24 bp, NAT#102 STM primer
ccatagcgatatctaccccaatct

SEQ ID NO: 376 - DNA, 24 bp, STM common primer
gcatgccctgcccctaagaattcg

SEQ ID NO: 377 - DNA, 18 bp, CNAG_03018 5 flanking region primer 1
agccgtttgtcattctgc

SEQ ID NO: 378 - DNA, 37 bp, CNAG_03018 5 flanking region primer 2
tcactggccgtcgttttacgtcgttgctcattttgcg

SEQ ID NO: 379 - DNA, 39 bp, CNAG_03018 3 flanking region primer 1
catggtcatagctgtttcctggcgaacctccaataaagc

SEQ ID NO: 380 - DNA, 18 bp, CNAG_03018 3 flanking region primer 2
cccttttttccctgcttc

SEQ ID NO: 381 - DNA, 18 bp, CNAG_03018 diagnostic screening primer, pairing with B79
aatagggatgccaaccag

SEQ ID NO: 382 - DNA, 18 bp, CNAG_03018 Southern blot probe primer
caaaaagtgtcagcacgc

SEQ ID NO: 383 - DNA, 20 bp, NAT#150 STM primer
acatacacccccatcccccc

SEQ ID NO: 384 - DNA, 24 bp, STM common primer
gcatgccctgcccctaagaattcg

SEQ ID NO: 385 - DNA, 20 bp, CNAG_01708 5 flanking region primer 1
ccgactcgttcgtctatctg

SEQ ID NO: 386 - DNA, 41 bp, CNAG_01708 5 flanking region primer 2
tcactggccgtcgttttactggagaggatagatgtgatgac

SEQ ID NO: 387 - DNA, 41 bp, CNAG_01708 3 flanking region primer 1
catggtcatagctgtttcctgaacttctacccaggtcgtgc

SEQ ID NO: 388 - DNA, 18 bp, CNAG_01708 3 flanking region primer 2
aactgcccttcttcaagc

SEQ ID NO: 389 - DNA, 20 bp, CNAG_01708 diagnostic screening primer, pairing with B79
tagcctctcccaatgtccac

SEQ ID NO: 390 - DNA, 20 bp, CNAG_01708 Southern blot probe primer
cgattctcctttgctgagtc

SEQ ID NO: 391 - DNA, 21 bp, NAT#159 STM primer
acgcaccagacacacaaccag

SEQ ID NO: 392 - DNA, 24 bp, STM common primer
gcatgccctgcccctaagaattcg

SEQ ID NO: 393 - DNA, 19 bp, CNAG_05861 5 flanking region primer 1
ggttttggtcacttcaccg

SEQ ID NO: 394 - DNA, 38 bp, CNAG_05861 5 flanking region primer 2
tcactggccgtcgttttacagcagaaaggagatgatgc

SEQ ID NO: 395 - DNA, 40 bp, CNAG_05861 3 flanking region primer 1
catggtcatagctgtttcctggacgacttttacgaccagg

SEQ ID NO: 396 - DNA, 18 bp, CNAG_05861 3 flanking region primer 2
aaatggaacaagcccgtc

SEQ ID NO: 397 - DNA, 18 bp, CNAG_05861 diagnostic screening primer, pairing with B79
tctgaagggcgtaaatgc

SEQ ID NO: 398 - DNA, 18 bp, CNAG_05861 Southern blot probe primer
aaggaatgggttgttggg

SEQ ID NO: 399 - DNA, 24 bp, NAT#184 STM primer
atatatggctcgagctagatagag

SEQ ID NO: 400 - DNA, 24 bp, STM common primer
gcatgccctgcccctaagaattcg

SEQ ID NO: 401 - DNA, 20 bp, CNAG_02066 5 flanking region primer 1
ccccattgtaaacattggtg

SEQ ID NO: 402 - DNA, 36 bp, CNAG_02066 5 flanking region primer 2
ctggccgtcgttttaccgtgatgtggagttgattcg

SEQ ID NO: 403 - DNA, 36 bp, CNAG_02066 3 flanking region primer 1
gtcatagctgtttcctgtgctgccaatggaaggttc

SEQ ID NO: 404 - DNA, 20 bp, CNAG_02066 3 flanking region primer 2
atagtctcgctccttggtgc

SEQ ID NO: 405 - DNA, 19 bp, CNAG_02066 diagnostic screening primer, pairing with B79
gttcgttatccgctctttg

SEQ ID NO: 406 - DNA, 19 bp, CNAG_02066 Southern blot probe primer
acataggcgagacagttgc

SEQ ID NO: 407 - DNA, 20 bp, NAT#191 STM primer
atatggatgtttttagcgag

SEQ ID NO: 408 - DNA, 24 bp, STM common primer
gcatgccctgcccctaagaattcg

SEQ ID NO: 409 - DNA, 19 bp, CNAG_03527 5 flanking region primer 1
ccatctcacggttgatacg

SEQ ID NO: 410 - DNA, 35 bp, CNAG_03527 5 flanking region primer 2
ctggccgtcgttttactcaaacccttatcccaccg

SEQ ID NO: 411 - DNA, 37 bp, CNAG_03527 3 flanking region primer 1
gtcatagctgtttcctgtctttccctgctttgcctgc

SEQ ID NO: 412 - DNA, 20 bp, CNAG_03527 3 flanking region primer 2
cgtcatccgtcgtgtaactg

SEQ ID NO: 413 - DNA, 19 bp, CNAG_03527 diagnostic screening primer, pairing with B79
tctcgcaaggtcagagttc

SEQ ID NO: 414 - DNA, 21 bp, CNAG_03527 Southern blot probe primer
ctatgagcgacattcacagac

SEQ ID NO: 415 - DNA, 20 bp, NAT#204 STM primer
gatctctcgcgcttggggga

SEQ ID NO: 416 - DNA, 24 bp, STM common primer
gcatgccctgcccctaagaattcg

SEQ ID NO: 417 - DNA, 18 bp, CNAG_04263 5 flanking region primer 1
tgtttccacacaccgatg

SEQ ID NO: 418 - DNA, 36 bp, CNAG_04263 5 flanking region primer 2
ctggccgtcgttttacggtggtggtcatctgtatgc

SEQ ID NO: 419 - DNA, 37 bp, CNAG_04263 3 flanking region primer 1
gtcatagctgtttcctgagaagatggagacgcacacg

SEQ ID NO: 420 - DNA, 19 bp, CNAG_04263 3 flanking region primer 2
gctattgcgtgaagactcc

SEQ ID NO: 421 - DNA, 20 bp, CNAG_04263 diagnostic screening primer, pairing with B79
cgtgattgagagtagcaacc

SEQ ID NO: 422 - DNA, 19 bp, CNAG_04263 Southern blot probe primer
gtaatgtcagtgagtgcgg

SEQ ID NO: 423 - DNA, 24 bp, NAT#205 STM primer
tatccccctctccgctctctagca

SEQ ID NO: 424 - DNA, 24 bp, STM common primer
gcatgccctgcccctaagaattcg

SEQ ID NO: 425 - DNA, 20 bp, CNAG_00018 5 flanking region primer 1
tttgcctcaatctctctcag

SEQ ID NO: 426 - DNA, 41 bp, CNAG_00018 5 flanking region primer 2
gctcactggccgtcgttttacggaatacaacatccacctcc

SEQ ID NO: 427 - DNA, 42 bp, CNAG_00018 3 flanking region primer 1
catggtcatagctgtttcctggcacgggttacattctacatc

SEQ ID NO: 428 - DNA, 20 bp, CNAG_00018 3 flanking region primer 2
ggggaggacttgaacttgag

SEQ ID NO: 429 - DNA, 18 bp, CNAG_00018 diagnostic screening primer, pairing with B79
aacaaactgccttcctcc

SEQ ID NO: 430 - DNA, 19 bp, CNAG_00018 Southern blot probe primer
gcttggtcggataaagatg

SEQ ID NO: 431 - DNA, 20 bp, NAT#211 STM primer
gcggtcgctttatagcgatt

SEQ ID NO: 432 - DNA, 24 bp, STM common primer
gcatgccctgcccctaagaattcg

SEQ ID NO: 433 - DNA, 19 bp, CNAG_05176 5 flanking region primer 1
tgagaaggaggatggtcac

SEQ ID NO: 434 - DNA, 37 bp, CNAG_05176 5 flanking region primer 2
tcactggccgtcgttttacatgtggatagtgttgcgg

SEQ ID NO: 435 - DNA, 40 bp, CNAG_05176 3 flanking region primer 1
catggtcatagctgtttcctggcaaaaagggagaatgtcg

SEQ ID NO: 436 - DNA, 19 bp, CNAG_05176 3 flanking region primer 2
tcatacagccgagttgacc

SEQ ID NO: 437 - DNA, 19 bp, CNAG_05176 diagnostic screening primer, pairing with B79
tgtgagtatgcctatcccg

SEQ ID NO: 438 - DNA, 19 bp, CNAG_05176 Southern blot probe primer
tcaccgagactaatggcac

SEQ ID NO: 439 - DNA, 20 bp, NAT#211 STM primer
gcggtcgctttatagcgatt

SEQ ID NO: 440 - DNA, 24 bp, STM common primer
gcatgccctgcccctaagaattcg

SEQ ID NO: 441 - DNA, 19 bp, CNAG_06339 5 flanking region primer 1
tagtgaaagactcggcacc

SEQ ID NO: 442 - DNA, 37 bp, CNAG_06339 5 flanking region primer 2
tcactggccgtcgttttaccagtcaccgcaaagattc

SEQ ID NO: 443 - DNA, 41 bp, CNAG_06339 3 flanking region primer 1
catggtcatagctgtttcctgcgcttcgttattacctgttc

SEQ ID NO: 444 - DNA, 22 bp, CNAG_06339 3 flanking region primer 2
ctccaggataagtagtgtgagg

SEQ ID NO: 445 - DNA, 20 bp, CNAG_06339 diagnostic screening primer, pairing with B79
gggaaagtagggtaaccacc

SEQ ID NO: 446 - DNA, 20 bp, CNAG_06339 Southern blot probe primer
gaggagaggtgaataatgcc

SEQ ID NO: 447 - DNA, 24 bp, NAT#213 STM primer
ctggggattttgatgtgtctatgt

SEQ ID NO: 448 - DNA, 24 bp, STM common primer
gcatgccctgcccctaagaattcg

SEQ ID NO: 449 - DNA, 19 bp, CNAG_07593 5 flanking region primer 1
gattgcttggatggacttc

SEQ ID NO: 450 - DNA, 39 bp, CNAG_07593 5 flanking region primer 2
tcactggccgtcgttttactgcctttcttgccgaactcg

SEQ ID NO: 451 - DNA, 40 bp, CNAG_07593 3 flanking region primer 1
catggtcatagctgtttcctgtttgaaggaccaggagcag

SEQ ID NO: 452 - DNA, 19 bp, CNAG_07593 3 flanking region primer 2
tcaagtgacacagtgccac

SEQ ID NO: 453 - DNA, 19 bp, CNAG_07593 diagnostic screening primer, pairing with B79
ccataatcagacagcgttg

SEQ ID NO: 454 - DNA, 19 bp, CNAG_07593 Southern blot probe primer
ggtttgggggaatagtgag

SEQ ID NO: 455 - DNA, 20 bp, NAT#218 STM primer
ctccacatccatcgctccaa

SEQ ID NO: 456 - DNA, 24 bp, STM common primer
gcatgccctgcccctaagaattcg

SEQ ID NO: 457 - DNA, 20 bp, CNAG_00670 5 flanking region primer 1
tgatgaagatgctgatgagg

SEQ ID NO: 458 - DNA, 41 bp, CNAG_00670 5 flanking region primer 2
gctcactggccgtcgttttactcatttggcgtctcacttac

SEQ ID NO: 459 - DNA, 39 bp, CNAG_00670 3 flanking region primer 1
catggtcatagctgtttcctgtgtgaaaggggagtgatg

SEQ ID NO: 460 - DNA, 19 bp, CNAG_00670 3 flanking region primer 2
agaatacatcgtggttggc

SEQ ID NO: 461 - DNA, 22 bp, CNAG_00670 diagnostic screening primer, pairing with B79
ggaagtgtagagtcaggagatg

SEQ ID NO: 462 - DNA, 21 bp, CNAG_00670 Southern blot probe primer
ggatgaaaggtgaaaggacac

SEQ ID NO: 463 - DNA, 19 bp, NAT#224 STM primer
aacctttaaatgggtagag

SEQ ID NO: 464 - DNA, 24 bp, STM common primer
gcatgccctgcccctaagaattcg

SEQ ID NO: 465 - DNA, 18 bp, CNAG_05010 5 flanking region primer 1
tccttcctttctaagccg

SEQ ID NO: 466 - DNA, 41 bp, CNAG_05010 5 flanking region primer 2
gctcactggccgtcgttttactgtcccctacttttactccg

SEQ ID NO: 467 - DNA, 41 bp, CNAG_05010 3 flanking region primer 1
catggtcatagctgtttcctgtgagggtttgataccttgtg

SEQ ID NO: 468 - DNA, 18 bp, CNAG_05010 3 flanking region primer 2
aagagcaacatccgcaag

SEQ ID NO: 469 - DNA, 19 bp, CNAG_05010 diagnostic screening primer, pairing with B79
aacagccttgccttacagc

SEQ ID NO: 470 - DNA, 19 bp, CNAG_05010 Southern blot probe primer
agtggtgaagggctaaatg

SEQ ID NO: 471 - DNA, 19 bp, NAT#224 STM primer
aacctttaaatgggtagag

SEQ ID NO: 472 - DNA, 24 bp, STM common primer
gcatgccctgcccctaagaattcg

SEQ ID NO: 473 - DNA, 18 bp, CNAG_04345 5 flanking region primer 1
aaaaggcagtcgtcttcg

SEQ ID NO: 474 - DNA, 40 bp, CNAG_04345 5 flanking region primer 2
ctggccgtcgttttacccttttagatactcacacaagccc

SEQ ID NO: 475 - DNA, 36 bp, CNAG_04345 3 flanking region primer 1
gtcatagctgtttcctgttctgggatgacttcacgc

SEQ ID NO: 476 - DNA, 19 bp, CNAG_04345 3 flanking region primer 2
ttactgctcctggtttggg

SEQ ID NO: 477 - DNA, 18 bp, CNAG_04345 diagnostic screening primer, pairing with B79
cctgcttcacaaaatggc

SEQ ID NO: 478 - DNA, 22 bp, CNAG_04345 Southern blot probe primer
gagtagtggtgtcagtgtgatg

SEQ ID NO: 479 - DNA, 20 bp, NAT#225 STM primer
ccatagaactagctaaagca

SEQ ID NO: 480 - DNA, 24 bp, STM common primer
gcatgccctgcccctaagaattcg

SEQ ID NO: 481 - DNA, 19 bp, CNAG_02774 5 flanking region primer 1
ttgagccagcctaagcaag

SEQ ID NO: 482 - DNA, 35 bp, CNAG_02774 5 flanking region primer 2
ctggccgtcgttttactcttcttttctgcggtcac

SEQ ID NO: 483 - DNA, 36 bp, CNAG_02774 3 flanking region primer 1
gtcatagctgtttcctggcttgatttcttggaccac

SEQ ID NO: 484 - DNA, 19 bp, CNAG_02774 3 flanking region primer 2
cgagataagaagcaacgcc

SEQ ID NO: 485 - DNA, 19 bp, CNAG_02774 diagnostic screening primer, pairing with B79
tgccagccaacctaatctg

SEQ ID NO: 486 - DNA, 20 bp, CNAG_02774 Southern blot probe primer
gagaggcagggagataactc

SEQ ID NO: 487 - DNA, 20 bp, NAT#230 STM primer
atgtaggtagggtgataggt

SEQ ID NO: 488 - DNA, 24 bp, STM common primer
gcatgccctgcccctaagaattcg

SEQ ID NO: 489 - DNA, 20 bp, CNAG_06425 5 flanking region primer 1
ctttcacgaacgcttgattc

SEQ ID NO: 490 - DNA, 35 bp, CNAG_06425 5 flanking region primer 2
ctggccgtcgttttacttggacagtttttcggcgg

SEQ ID NO: 491 - DNA, 36 bp, CNAG_06425 3 flanking region primer 1
gtcatagctgtttcctgatgtgcctgcggatttctc

SEQ ID NO: 492 - DNA, 19 bp, CNAG_06425 3 flanking region primer 2
tgagaccgctgaaagttcc

SEQ ID NO: 493 - DNA, 19 bp, CNAG_06425 diagnostic screening primer, pairing with B79
taatcgccgacaaagggtg

SEQ ID NO: 494 - DNA, 18 bp, CNAG_06425 Southern blot probe primer
ccctttttttgtgcgacc

SEQ ID NO: 495 - DNA, 24 bp, NAT#288 STM primer
ctatccaactagacctctagctac

SEQ ID NO: 496 - DNA, 24 bp, STM common primer
gcatgccctgcccctaagaattcg

SEQ ID NO: 497 - DNA, 22 bp, CNAG_05255 5 flanking region primer 1
atggtcaccgtcacaaggaagc

SEQ ID NO: 498 - DNA, 40 bp, CNAG_05255 5 flanking region primer 2
ctggccgtcgttttactacacattcggcttggttgcggac

SEQ ID NO: 499 - DNA, 38 bp, CNAG_05255 3 flanking region primer 1
gtcatagctgtttcctgcgaggtttgtatcccagtcag

SEQ ID NO: 500 - DNA, 20 bp, CNAG_05255 3 flanking region primer 2
aggggctatctctgcttcac

SEQ ID NO: 501 - DNA, 24 bp, CNAG_05255 diagnostic screening primer, pairing with B79
ttctgtgcccacctctactctcag

SEQ ID NO: 502 - DNA, 20 bp, CNAG_05255 Southern blot probe primer
accaaaactcgtcgtaggcg

SEQ ID NO: 503 - DNA, 24 bp, NAT#288 STM primer
ctatccaactagacctctagctac

SEQ ID NO: 504 - DNA, 24 bp, STM common primer
gcatgccctgcccctaagaattcg

SEQ ID NO: 505 - DNA, 19 bp, CNAG_05049 5 flanking region primer 1
atcaggacgagtggcattg

SEQ ID NO: 506 - DNA, 39 bp, CNAG_05049 5 flanking region primer 2
tcactggccgtcgttttacgagtcttctttgggcatagc

SEQ ID NO: 507 - DNA, 40 bp, CNAG_05049 3 flanking region primer 1
catggtcatagctgtttcctgagtggatgatgaggactcg

SEQ ID NO: 508 - DNA, 21 bp, CNAG_05049 3 flanking region primer 2
gtttcctatcttcagtcggag

SEQ ID NO: 509 - DNA, 20 bp, CNAG_05049 diagnostic screening primer, pairing with B79
gatagcagaggagaaaaggc

SEQ ID NO: 510 - DNA, 18 bp, CNAG_05049 Southern blot probe primer
tatttggggttgaggctg

SEQ ID NO: 511 - DNA, 20 bp, NAT#123 STM primer
ctatcgaccaaccaacacag

SEQ ID NO: 512 - DNA, 24 bp, STM common primer
gcatgccctgcccctaagaattcg

SEQ ID NO: 513 - DNA, 18 bp, CNAG_05222 5 flanking region primer 1
gagggtcctttggttttg

SEQ ID NO: 514 - DNA, 37 bp, CNAG_05222 5 flanking region primer 2
tcactggccgtcgttttactttcacactcacggttgg

SEQ ID NO: 515 - DNA, 39 bp, CNAG_05222 3 flanking region primer 1
catggtcatagctgtttcctggttgccccttttgacaag

SEQ ID NO: 516 - DNA, 19 bp, CNAG_05222 3 flanking region primer 2
aacttacggcgacaacaac

SEQ ID NO: 517 - DNA, 18 bp, CNAG_05222 diagnostic screening primer, pairing with B79
tccacataatagccaccg

SEQ ID NO: 518 - DNA, 20 bp, CNAG_05222 Southern blot probe primer
gctatgttcaggagcgatac

SEQ ID NO: 519 - DNA, 20 bp, NAT#123 STM primer
ctatcgaccaaccaacacag

SEQ ID NO: 520 - DNA, 24 bp, STM common primer
gcatgccctgcccctaagaattcg

SEQ ID NO: 521 - DNA, 18 bp, CNAG_04130 5 flanking region primer 1
cattgacgccatagcaag

SEQ ID NO: 522 - DNA, 38 bp, CNAG_04130 5 flanking region primer 2
tcactggccgtcgttttacgtgtttggaatgcggtttc

SEQ ID NO: 523 - DNA, 41 bp, CNAG_04130 3 flanking region primer 1
catggtcatagctgtttcctgtggatgaggttgaggggaac

SEQ ID NO: 524 - DNA, 21 bp, CNAG_04130 3 flanking region primer 2
gtagtgtaagggcaggaagag

SEQ ID NO: 525 - DNA, 21 bp, CNAG_04130 diagnostic screening primer, pairing with B79
ttctactcataagggctacgc

SEQ ID NO: 526 - DNA, 21 bp, CNAG_04130 Southern blot probe primer
ttctactcataagggctacgc

SEQ ID NO: 527 - DNA, 19 bp, CNAG_00193 5 flanking region primer 1
gggcagaaatagttggcag

SEQ ID NO: 528 - DNA, 34 bp, CNAG_00193 5 flanking region primer 2
ctggccgtcgttttactttttccccccgatgtag

SEQ ID NO: 529 - DNA, 36 bp, CNAG_00193 3 flanking region primer 1
gtcatagctgtttcctgttcccgcaagaacagtgtc

SEQ ID NO: 530 - DNA, 20 bp, CNAG_00193 3 flanking region primer 2
ttcaggatgtccaaactcag

SEQ ID NO: 531 - DNA, 19 bp, CNAG_00193 diagnostic screening primer, pairing with B79
aaggggtaagaaatcgggc

SEQ ID NO: 532 - DNA, 19 bp, CNAG_00193 Southern blot probe primer
tgctgagagacagggaatc

SEQ ID NO: 533 - DNA, 20 bp, NAT#227 STM primer
tcgtggtttagagggagcgc

SEQ ID NO: 534 - DNA, 24 bp, STM common primer
gcatgccctgcccctaagaattcg

SEQ ID NO: 535 - DNA, 20 bp, CNAG_02700 5 flanking region primer 1
tgaaatcagactccagcctc

SEQ ID NO: 536 - DNA, 38 bp, CNAG_02700 5 flanking region primer 2
tcactggccgtcgttttacgcgaccacatttacactcg

SEQ ID NO: 537 - DNA, 41 bp, CNAG_02700 3 flanking region primer 1
catggtcatagctgtttcctggccacagaacaataactggg

SEQ ID NO: 538 - DNA, 19 bp, CNAG_02700 3 flanking region primer 2
gcgtatgaataagcgttgg

SEQ ID NO: 539 - DNA, 18 bp, CNAG_02700 diagnostic screening primer, pairing with B79
agcaaaacagaagcagcg

SEQ ID NO: 540 - DNA, 18 bp, CNAG_02700 Southern blot probe primer
agaaagcagcatttgggg

SEQ ID NO: 541 - DNA, 20 bp, NAT#230 STM primer
atgtaggtagggtgataggt

SEQ ID NO: 542 - DNA, 24 bp, STM common primer
gcatgccctgcccctaagaattcg

SEQ ID NO: 543 - DNA, 19 bp, CNAG_04586 5 flanking region primer 1
tccatctcccaatccacag

SEQ ID NO: 544 - DNA, 38 bp, CNAG_04586 5 flanking region primer 2
tcactggccgtcgttttacgcttgattaggcggataag

SEQ ID NO: 545 - DNA, 41 bp, CNAG_04586 3 flanking region primer 1
catggtcatagctgtttcctgtggacgaaaagacccctacc

SEQ ID NO: 546 - DNA, 18 bp, CNAG_04586 3 flanking region primer 2
aacactggaatgtgcgtg

SEQ ID NO: 547 - DNA, 20 bp, CNAG_04586 diagnostic screening primer, pairing with B79
ttggtggtgcggttttgtgc

SEQ ID NO: 548 - DNA, 18 bp, CNAG_04586 Southern blot probe primer
tgatgttggttcgtgacc

SEQ ID NO: 549 - DNA, 21 bp, NAT#159 STM primer
acgcaccagacacacaaccag

SEQ ID NO: 550 - DNA, 24 bp, STM common primer
gcatgccctgcccctaagaattcg

SEQ ID NO: 551 - DNA, 18 bp, CNAG_05153 5 flanking region primer 1
aaaaccaagtggaacccg

SEQ ID NO: 552 - DNA, 35 bp, CNAG_05153 5 flanking region primer 2
ctggccgtcgttttactggttgacgctgttagcac

SEQ ID NO: 553 - DNA, 37 bp, CNAG_05153 3 flanking region primer 1
gtcatagctgtttcctgataggcaggctggtggaaac

SEQ ID NO: 554 - DNA, 19 bp, CNAG_05153 3 flanking region primer 2
accacatttgcttccgagc

SEQ ID NO: 555 - DNA, 21 bp, CNAG_05153 diagnostic screening primer, pairing with JOHE12579
tggctgaactgtaggttagtg

SEQ ID NO: 556 - DNA, 18 bp, CNAG_05153 Southern blot probe primer
cggcgataaggtttttgc

SEQ ID NO: 557 - DNA, 24 bp, NAT#290 STM primer
accgacagctcgaacaagcaagag

SEQ ID NO: 558 - DNA, 24 bp, STM common primer
gcatgccctgcccctaagaattcg

SEQ ID NO: 559 - DNA, 20 bp, CNAG_02723 5 flanking region primer 1
gcttccttatcggtagggac

SEQ ID NO: 560 - DNA, 39 bp, CNAG_02723 5 flanking region primer 2
tcactggccgtcgttttacgactggacattgacgaagac

SEQ ID NO: 561 - DNA, 40 bp, CNAG_02723 3 flanking region primer 1
catggtcatagctgtttcctgtggtgacagtgacgcttac

SEQ ID NO: 562 - DNA, 19 bp, CNAG_02723 3 flanking region primer 2
attgtcaggatgtgggttc

SEQ ID NO: 563 - DNA, 21 bp, CNAG_02723 diagnostic screening primer, pairing with B79
gcttactcccaaactcacacc

SEQ ID NO: 564 - DNA, 18 bp, CNAG_02723 Southern blot probe primer
atggatttggcagaacgg

SEQ ID NO: 565 - DNA, 24 bp, NAT#201 STM primer
caccctctatctcgagaaagctcc

SEQ ID NO: 566 - DNA, 24 bp, STM common primer
gcatgccctgcccctaagaattcg

SEQ ID NO: 567 - DNA, 19 bp, CNAG_03741 5 flanking region primer 1
gccgtctcctgatgtaatc

SEQ ID NO: 568 - DNA, 36 bp, CNAG_03741 5 flanking region primer 2
ctggccgtcgttttaccgactgtcatcaacgactgg

SEQ ID NO: 569 - DNA, 36 bp, CNAG_03741 3 flanking region primer 1
ctggccgtcgttttacgcgtcaacaggaataaaacc

SEQ ID NO: 570 - DNA, 22 bp, CNAG_03741 3 flanking region primer 2
ctgtgcctttctccaagataag

SEQ ID NO: 571 - DNA, 22 bp, CNAG_03741 diagnostic screening primer, pairing with B79
ggataagcagaacatagttgcg

SEQ ID NO: 572 - DNA, 21 bp, CNAG_03741 Southern blot probe primer
tctcttcttcttctgacctgc

SEQ ID NO: 573 - DNA, 24 bp, NAT#273 STM primer
gagatctttcgggaggtctggatt

SEQ ID NO: 574 - DNA, 24 bp, STM common primer
gcatgccctgcccctaagaattcg

SEQ ID NO: 575 - DNA, 18 bp, CNAG_07411 5 flanking region primer 1
agacccgccaaaacaatc

SEQ ID NO: 576 - DNA, 35 bp, CNAG_07411 5 flanking region primer 2
ctggccgtcgttttacttggacctacgctgacttc

SEQ ID NO: 577 - DNA, 37 bp, CNAG_07411 3 flanking region primer 1
gtcatagctgtttcctggacttgcgttctgattttgg

SEQ ID NO: 578 - DNA, 20 bp, CNAG_07411 3 flanking region primer 2
gctgttatcaagagaatgcc

SEQ ID NO: 579 - DNA, 19 bp, CNAG_07411 diagnostic screening primer, pairing with B79
acgactggctatcaagcag

SEQ ID NO: 580 - DNA, 19 bp, CNAG_07411 Southern blot probe primer
tacgaggattgagtctggc

SEQ ID NO: 581 - DNA, 24 bp, NAT#288 STM primer
ctatccaactagacctctagctac

SEQ ID NO: 582 - DNA, 24 bp, STM common primer
gcatgccctgcccctaagaattcg

SEQ ID NO: 583 - DNA, 20 bp, CNAG_03849 5 flanking region primer 1
tagtggttcccgtttgtgcg

SEQ ID NO: 584 - DNA, 40 bp, CNAG_03849 5 flanking region primer 2
gctcactggccgtcgttttaccttacgcctttttccatcg

SEQ ID NO: 585 - DNA, 41 bp, CNAG_03849 3 flanking region primer 1
catggtcatagctgtttcctgtcaaacggcgattggtggtc

SEQ ID NO: 586 - DNA, 20 bp, CNAG_03849 3 flanking region primer 2
tggtgaaggggaagattggg

SEQ ID NO: 587 - DNA, 19 bp, CNAG_03849 diagnostic screening primer, pairing with B79
aacaagccgaggaatgagg

SEQ ID NO: 588 - DNA, 19 bp, CNAG_03849 Southern blot probe primer
tgagtgaacgaagagtgcc

SEQ ID NO: 589 - DNA, 20 bp, NAT#6 STM primer
atagctaccacacgatagct

SEQ ID NO: 590 - DNA, 24 bp, STM common primer
gcatgccctgcccctaagaattcg

SEQ ID NO: 591 - DNA, 19 bp, CNAG_04916 5 flanking region primer 1
ttgcgttgagacatcactg

SEQ ID NO: 592 - DNA, 43 bp, CNAG_04916 5 flanking region primer 2
gctcactggccgtcgttttacgctcctatgttaccaatgttgc

SEQ ID NO: 593 - DNA, 40 bp, CNAG_04916 3 flanking region primer 1
catggtcatagctgtttcctgacccatttgctttcctggc

SEQ ID NO: 594 - DNA, 20 bp, CNAG_04916 3 flanking region primer 2
tctcaacgagtcgctttcgc

SEQ ID NO: 595 - DNA, 20 bp, CNAG_04916 diagnostic screening primer, pairing with B79
aaaagcatcctgcccagcac

SEQ ID NO: 596 - DNA, 20 bp, CNAG_04916 Southern blot probe primer
gttgaaagtagttgcgttgg

SEQ ID NO: 597 - DNA, 20 bp, NAT#212 STM primer
agagcgatcgcgttatagat

SEQ ID NO: 598 - DNA, 24 bp, STM common primer
gcatgccctgcccctaagaattcg

SEQ ID NO: 599 - DNA, 19 bp, CNAG_04012 5 flanking region primer 1
ttggtggagtgattgaccc

SEQ ID NO: 600 - DNA, 36 bp, CNAG_04012 5 flanking region primer 2
ctggccgtcgttttacaatcaaaccagaaggagagc

SEQ ID NO: 601 - DNA, 39 bp, CNAG_04012 3 flanking region primer 1
gtcatagctgtttcctgaggaggataaaggaagagagtg

SEQ ID NO: 602 - DNA, 19 bp, CNAG_04012 3 flanking region primer 2
ttatgctggtggtgcctac

SEQ ID NO: 603 - DNA, 19 bp, CNAG_04012 diagnostic screening primer, pairing with B79
accgaagaggatgaggttg

SEQ ID NO: 604 - DNA, 20 bp, CNAG_04012 Southern blot probe primer
cagtggtggttgagattgac

SEQ ID NO: 605 - DNA, 20 bp, NAT#212 STM primer
agagcgatcgcgttatagat

SEQ ID NO: 606 - DNA, 24 bp, STM common primer
gcatgccctgcccctaagaattcg

SEQ ID NO: 607 - DNA, 20 bp, CNAG_04090 5 flanking region primer 1
gagtagaggagtggattggg

SEQ ID NO: 608 - DNA, 39 bp, CNAG_04090 5 flanking region primer 2
gctcactggccgtcgttttacccattgttcaagcagagc

SEQ ID NO: 609 - DNA, 42 bp, CNAG_04090 3 flanking region primer 1
catggtcatagctgtttcctgggcttactgctatcttgatgc

SEQ ID NO: 610 - DNA, 24 bp, CNAG_04090 3 flanking region primer 2
gaaagaggaactacatactgggtc

SEQ ID NO: 611 - DNA, 20 bp, CNAG_04090 diagnostic screening primer, pairing with B79
gtcttttgctccttgaaacc

SEQ ID NO: 612 - DNA, 20 bp, CNAG_04090 Southern blot probe primer
accaggtgtaaacccagtcc

SEQ ID NO: 613 - DNA, 20 bp, NAT#220 STM primer
cagatctcgaacgataccca

SEQ ID NO: 614 - DNA, 24 bp, STM common primer
gcatgccctgcccctaagaattcg

SEQ ID NO: 615 - DNA, 21 bp, CNAG_05375 5 flanking region primer 1
ggaagcattactgtcccatag

SEQ ID NO: 616 - DNA, 43 bp, CNAG_05375 5 flanking region primer 2
gctcactggccgtcgttttacagaaacaggagagagagtagcc

SEQ ID NO: 617 - DNA, 39 bp, CNAG_05375 3 flanking region primer 1
catggtcatagctgtttcctgtcttggatttcaacgggg

SEQ ID NO: 618 - DNA, 20 bp, CNAG_05375 3 flanking region primer 2
gtagttccgttatttgctgg

SEQ ID NO: 619 - DNA, 22 bp, CNAG_05375 diagnostic screening primer, pairing with B79
ggttgaagatggacgagtagac

SEQ ID NO: 620 - DNA, 20 bp, CNAG_05375 Southern blot probe primer
cattcacctcccttagaagc

SEQ ID NO: 621 - DNA, 19 bp, NAT#224 STM primer
aacctttaaatgggtagag

SEQ ID NO: 622 - DNA, 24 bp, STM common primer
gcatgccctgcccctaagaattcg

SEQ ID NO: 623 - DNA, 20 bp, CNAG_07797 5 flanking region primer 1
agggagaacaccacaggatg

SEQ ID NO: 624 - DNA, 38 bp, CNAG_07797 5 flanking region primer 2
tcactggccgtcgttttacaggaatggaggtggtgaac

SEQ ID NO: 625 - DNA, 40 bp, CNAG_07797 3 flanking region primer 1
catggtcatagctgtttcctgggaaagtcagtgatgctcc

SEQ ID NO: 626 - DNA, 18 bp, CNAG_07797 3 flanking region primer 2
gctttcttccttttcccg

SEQ ID NO: 627 - DNA, 18 bp, CNAG_07797 diagnostic screening primer, pairing with B79
atcaatggtttcgtcggc

SEQ ID NO: 628 - DNA, 18 bp, CNAG_07797 Southern blot probe primer
ggggcgttgaaaatgatg

SEQ ID NO: 629 - DNA, 20 bp, NAT#231 STM primer
gagagatcccaacatcacgc

SEQ ID NO: 630 - DNA, 24 bp, STM common primer
gcatgccctgcccctaagaattcg

SEQ ID NO: 631 - DNA, 22 bp, CNAG_05538 5 flanking region primer 1
ggtctcaacaaagcacttactg

SEQ ID NO: 632 - DNA, 40 bp, CNAG_05538 5 flanking region primer 2
tcactggccgtcgttttacgtaatagtcaggcggtttctc

SEQ ID NO: 633 - DNA, 41 bp, CNAG_05538 3 flanking region primer 1
catggtcatagctgtttcctgagttaccagaggaggagtgg

SEQ ID NO: 634 - DNA, 20 bp, CNAG_05538 3 flanking region primer 2
gattctctttaccctcagcc

SEQ ID NO: 635 - DNA, 20 bp, CNAG_05538 diagnostic screening primer, pairing with B79
tccgattctattgactctgc

SEQ ID NO: 636 - DNA, 20 bp, CNAG_05538 Southern blot probe primer
gtatcatccattttcctggc

SEQ ID NO: 637 - DNA, 20 bp, NAT#240 STM primer
ggtgttggatcggggtggat

SEQ ID NO: 638 - DNA, 24 bp, STM common primer
gcatgccctgcccctaagaattcg

SEQ ID NO: 639 - DNA, 18 bp, CNAG_00332 5 flanking region primer 1
tgattgtcgtccttgtgg

SEQ ID NO: 640 - DNA, 39 bp, CNAG_00332 5 flanking region primer 2
gctcactggccgtcgttttactttgcgtgactgttctgc

SEQ ID NO: 641 - DNA, 42 bp, CNAG_00332 3 flanking region primer 1
catggtcatagctgtttcctgcggtttgcgaagatacagaac

SEQ ID NO: 642 - DNA, 18 bp, CNAG_00332 3 flanking region primer 2
tatggatgcgtgggaatg

SEQ ID NO: 643 - DNA, 18 bp, CNAG_00332 diagnostic screening primer, pairing with B79
gccagaccaatcaaatgc

SEQ ID NO: 644 - DNA, 19 bp, CNAG_00332 Southern blot probe primer
gaagaagggttgaatgtcg

SEQ ID NO: 645 - DNA, 24 bp, NAT#290 STM primer
accgacagctcgaacaagcaagag

SEQ ID NO: 646 - DNA, 24 bp, STM common primer
gcatgccctgcccctaagaattcg

SEQ ID NO: 647 - DNA, 19 bp, CNAG_04023 5 flanking region primer 1
agcaggatagacagcgaag

SEQ ID NO: 648 - DNA, 35 bp, CNAG_04023 5 flanking region primer 2
ctggccgtcgttttactgtccttgataggtcggag

SEQ ID NO: 649 - DNA, 35 bp, CNAG_04023 3 flanking region primer 1
gtcatagctgtttcctgtggaacacattggaggag

SEQ ID NO: 650 - DNA, 18 bp, CNAG_04023 3 flanking region primer 2
aatgggtgtatgatggcg

SEQ ID NO: 651 - DNA, 19 bp, CNAG_04023 diagnostic screening primer, pairing with B79
cagaacgcattgtttgtgc

SEQ ID NO: 652 - DNA, 19 bp, CNAG_04023 Southern blot probe primer
gtagtaaacgccttgagcc

SEQ ID NO: 653 - DNA, 20 bp, CNAG_05311 5 flanking region primer 1
caacaagttccatcacatcg

SEQ ID NO: 654 - DNA, 40 bp, CNAG_05311 5 flanking region primer 2
gctcactggccgtcgttttacgggtaaaacctggcttagg

SEQ ID NO: 655 - DNA, 39 bp, CNAG_05311 3 flanking region primer 1
catggtcatagctgtttcctgggatttggatgaacctgg

SEQ ID NO: 656 - DNA, 21 bp, CNAG_05311 3 flanking region primer 2
gagaaagaggtttgtcgtgag

SEQ ID NO: 657 - DNA, 18 bp, CNAG_05311 diagnostic screening primer, pairing with B79
ttctactttccgccaagg

SEQ ID NO: 658 - DNA, 19 bp, CNAG_05311 Southern blot probe primer
gagatgggtcactaatcgc

SEQ ID NO: 659 - DNA, 19 bp, CNAG_03086 5 flanking region primer 1
aatctcctttgcccgactc

SEQ ID NO: 660 - DNA, 38 bp, CNAG_03086 5 flanking region primer 2
tcactggccgtcgttttacataccttgtctttgcgggc

SEQ ID NO: 661 - DNA, 41 bp, CNAG_03086 3 flanking region primer 1
catggtcatagctgtttcctgattgaaggtggcagtagatg

SEQ ID NO: 662 - DNA, 18 bp, CNAG_03086 3 flanking region primer 2
aaaatgtgggcggatgag

SEQ ID NO: 663 - DNA, 19 bp, CNAG_03086 diagnostic screening primer, pairing with B79
tcagtcgggaagagtttgc

SEQ ID NO: 664 - DNA, 19 bp, CNAG_03086 Southern blot probe primer
aggcgagagtaagaatgcg

SEQ ID NO: 665 - DNA, 20 bp, NAT#191 STM primer
atatggatgtttttagcgag

SEQ ID NO: 666 - DNA, 24 bp, STM common primer
gcatgccctgcccctaagaattcg

SEQ ID NO: 667 - DNA, 18 bp, CNAG_03336 5 flanking region primer 1
gtgccttattccaatggg

SEQ ID NO: 668 - DNA, 34 bp, CNAG_03336 5 flanking region primer 2
ctggccgtcgttttacttcttgctgcctgtttgg

SEQ ID NO: 669 - DNA, 35 bp, CNAG_03336 3 flanking region primer 1
ctggccgtcgttttacccaacaataatcacgcagg

SEQ ID NO: 670 - DNA, 20 bp, CNAG_03336 3 flanking region primer 2
ccatcctttttttagcggtc

SEQ ID NO: 671 - DNA, 19 bp, CNAG_03336 diagnostic screening primer, pairing with B79
cgaggtgattgatgtgagc

SEQ ID NO: 672 - DNA, 20 bp, CNAG_03336 Southern blot probe primer
ttcaagagcggactggacag

SEQ ID NO: 673 - DNA, 20 bp, NAT#204 STM primer
gatctctcgcgcttggggga

SEQ ID NO: 674 - DNA, 24 bp, STM common primer
gcatgccctgcccctaagaattcg

SEQ ID NO: 675 - DNA, 19 bp, CNAG_03229 5 flanking region primer 1
gtgggttactttgggtgag

SEQ ID NO: 676 - DNA, 37 bp, CNAG_03229 5 flanking region primer 2
tcactggccgtcgttttacaaaagggacttgctgtcg

SEQ ID NO: 677 - DNA, 40 bp, CNAG_03229 3 flanking region primer 1
catggtcatagctgtttcctggaaagaaaggaaatcgccg

SEQ ID NO: 678 - DNA, 18 bp, CNAG_03229 3 flanking region primer 2
tggaagatggtgacgaag

SEQ ID NO: 679 - DNA, 18 bp, CNAG_03229 diagnostic screening primer, pairing with B79
ttgcgatttccgactacc

SEQ ID NO: 680 - DNA, 18 bp, CNAG_03229 Southern blot probe primer
tggaggcgaataatggtc

SEQ ID NO: 681 - DNA, 20 bp, NAT#227 STM primer
tcgtggtttagagggagcgc

SEQ ID NO: 682 - DNA, 24 bp, STM common primer
gcatgccctgcccctaagaattcg

SEQ ID NO: 683 - DNA, 19 bp, CNAG_01883 5 flanking region primer 1
tactcgctgcttagggttc

SEQ ID NO: 684 - DNA, 35 bp, CNAG_01883 5 flanking region primer 2
ctggccgtcgttttacatggcatactccaggtctg

SEQ ID NO: 685 - DNA, 36 bp, CNAG_01883 3 flanking region primer 1
gtcatagctgtttcctgccctccatttacttctccg

SEQ ID NO: 686 - DNA, 22 bp, CNAG_01883 3 flanking region primer 2
tagcagtagggctcctgattcg

SEQ ID NO: 687 - DNA, 19 bp, CNAG_01883 diagnostic screening primer, pairing with B79
ttggaggtctttatcagcg

SEQ ID NO: 688 - DNA, 19 bp, CNAG_01883 Southern blot probe primer
ggagaagtaaatggagggg

SEQ ID NO: 689 - DNA, 24 bp, NAT#125 STM primer
cgctacagccagcgcgcgcaagcg

SEQ ID NO: 690 - DNA, 24 bp, STM common primer
gcatgccctgcccctaagaattcg

SEQ ID NO: 691 - DNA, 20 bp, CNAG_04837 5 flanking region primer 1
tgaaacagtgaatcaggcac

SEQ ID NO: 692 - DNA, 40 bp, CNAG_04837 5 flanking region primer 2
gctcactggccgtcgttttactcagtgtcaacggtcattg

SEQ ID NO: 693 - DNA, 42 bp, CNAG_04837 3 flanking region primer 1
catggtcatagctgtttcctggaaaggggtagggataagttg

SEQ ID NO: 694 - DNA, 20 bp, CNAG_04837 3 flanking region primer 2
actgaacgacaagagacgac

SEQ ID NO: 695 - DNA, 18 bp, CNAG_04837 diagnostic screening primer, pairing with B79
taagagaaaaggggctgc

SEQ ID NO: 696 - DNA, 21 bp, CNAG_04837 Southern blot probe primer 1
tgtccccatcaactctacaac

SEQ ID NO: 697 - DNA, 20 bp, CNAG_04837 Southern blot probe primer 2
cttctgctttcaccattagc

SEQ ID NO: 698 - DNA, 21 bp, NAT#146 STM primer
actagccccccctcaccacct

SEQ ID NO: 699 - DNA, 24 bp, STM common primer
gcatgccctgcccctaagaattcg

SEQ ID NO: 700 - DNA, 19 bp, CNAG_00514 5 flanking region primer 1
ggtgtttccatacgaaccg

SEQ ID NO: 701 - DNA, 38 bp, CNAG_00514 5 flanking region primer 2
ctggccgtcgttttacggagccatttcttacttatgcg

SEQ ID NO: 702 - DNA, 35 bp, CNAG_00514 3 flanking region primer 1
gtcatagctgtttcctgaatcccaaggaccatctg

SEQ ID NO: 703 - DNA, 20 bp, CNAG_00514 3 flanking region primer 2
gctgagaaggagaggatagc

SEQ ID NO: 704 - DNA, 20 bp, CNAG_00514 diagnostic screening primer, pairing with B79
gtggttgaaagtattaggcg

SEQ ID NO: 705 - DNA, 19 bp, CNAG_00514 Southern blot probe primer
gaggattggtgatggactg

SEQ ID NO: 706 - DNA, 24 bp, NAT#201 STM primer
caccctctatctcgagaaagctcc

SEQ ID NO: 707 - DNA, 24 bp, STM common primer
gcatgccctgcccctaagaattcg

SEQ ID NO: 708 - DNA, 20 bp, CNAG_03409 5 flanking region primer 1
cctcaccgattcattcactg

SEQ ID NO: 709 - DNA, 38 bp, CNAG_03409 5 flanking region primer 2
ctggccgtcgttttacttttctcccttcttcgcccgac

SEQ ID NO: 710 - DNA, 37 bp, CNAG_03409 3 flanking region primer 1
gtcatagctgtttcctgaggttcaagcccagactcag

SEQ ID NO: 711 - DNA, 20 bp, CNAG_03409 3 flanking region primer 2
agtatctacggtgctggtgc

SEQ ID NO: 712 - DNA, 20 bp, CNAG_03409 diagnostic screening primer, pairing with B79
tgaggatgatgactggggac

SEQ ID NO: 713 - DNA, 20 bp, CNAG_03409 Southern blot probe primer 1
acttccaatgctcaaccccg

SEQ ID NO: 714 - DNA, 20 bp, CNAG_03409 Southern blot probe primer 2
gcaggacaagaaggagagtg

SEQ ID NO: 715 - DNA, 24 bp, NAT#201 STM primer
caccctctatctcgagaaagctcc

SEQ ID NO: 716 - DNA, 24 bp, STM common primer
gcatgccctgcccctaagaattcg

SEQ ID NO: 717 - DNA, 19 bp, CNAG_05392 5 flanking region primer 1
aagttgtgaaaccaccagg

SEQ ID NO: 718 - DNA, 38 bp, CNAG_05392 5 flanking region primer 2
tcactggccgtcgttttactcaccctgtagatgtgtgg

SEQ ID NO: 719 - DNA, 42 bp, CNAG_05392 3 flanking region primer 1
catggtcatagctgtttcctgggagtccctgtgaagtaaaag

SEQ ID NO: 720 - DNA, 20 bp, CNAG_05392 3 flanking region primer 2
tgagccaaagtagcagtcag

SEQ ID NO: 721 - DNA, 19 bp, CNAG_05392 diagnostic screening primer, pairing with B79
gaatggaccttggaaaacg

SEQ ID NO: 722 - DNA, 20 bp, CNAG_05392 Southern blot probe primer
cggtctgtgtgcttcttcac

SEQ ID NO: 723 - DNA, 20 bp, NAT#204 STM primer
gatctctcgcgcttggggga

SEQ ID NO: 724 - DNA, 24 bp, STM common primer
gcatgccctgcccctaagaattcg

SEQ ID NO: 725 - DNA, 20 bp, CNAG_04895 5 flanking region primer 1
ttcgtagttagccagcagag

SEQ ID NO: 726 - DNA, 38 bp, CNAG_04895 5 flanking region primer 2
tcactggccgtcgttttacgttcttgatgtggaggagc

SEQ ID NO: 727 - DNA, 40 bp, CNAG_04895 3 flanking region primer 1
catggtcatagctgtttcctgcccaacccttatgcgtatg

SEQ ID NO: 728 - DNA, 18 bp, CNAG_04895 3 flanking region primer 2
agcgtctccctcaaaaac

SEQ ID NO: 729 - DNA, 18 bp, CNAG_04895 diagnostic screening primer, pairing with B79
ttagcgaccgaaaaaggg

SEQ ID NO: 730 - DNA, 19 bp, CNAG_04895 Southern blot probe primer
aagatgacgcagaactggg

SEQ ID NO: 731 - DNA, 20 bp, NAT#204 STM primer
gatctctcgcgcttggggga

SEQ ID NO: 732 - DNA, 24 bp, STM common primer
gcatgccctgcccctaagaattcg

SEQ ID NO: 733 - DNA, 19 bp, CNAG_04176 5 flanking region primer 1
ttgacacggggactaatcg

SEQ ID NO: 734 - DNA, 40 bp, CNAG_04176 5 flanking region primer 2
gctcactggccgtcgttttacgattagcccagtcttagcg

SEQ ID NO: 735 - DNA, 41 bp, CNAG_04176 3 flanking region primer 1
catggtcatagctgtttcctgagaagcagggagcaaaacgg

SEQ ID NO: 736 - DNA, 19 bp, CNAG_04176 3 flanking region primer 2
ccgaaaagttgagcaagac

SEQ ID NO: 737 - DNA, 23 bp, CNAG_04176 diagnostic screening primer, pairing with B79
cgatagcctttgtagtaggtctc

SEQ ID NO: 738 - DNA, 20 bp, CNAG_04176 Southern blot probe primer
gggatttgattatctggagg

SEQ ID NO: 739 - DNA, 24 bp, NAT#205 STM primer
tatccccctctccgctctctagca

SEQ ID NO: 740 - DNA, 24 bp, STM common primer
gcatgccctgcccctaagaattcg

SEQ ID NO: 741 - DNA, 19 bp, CNAG_07724 5 flanking region primer 1
caaagaaaacgctcactcc

SEQ ID NO: 742 - DNA, 40 bp, CNAG_07724 5 flanking region primer 2
tcactggccgtcgttttacggatagaacaagacaagagcg

SEQ ID NO: 743 - DNA, 41 bp, CNAG_07724 3 flanking region primer 1
catggtcatagctgtttcctgacttcagtcgttaccagcac

SEQ ID NO: 744 - DNA, 19 bp, CNAG_07724 3 flanking region primer 2
tctttgagcacatcaggtg

SEQ ID NO: 745 - DNA, 19 bp, CNAG_07724 diagnostic screening primer, pairing with B79
ccgtcattatcgtgtctcc

SEQ ID NO: 746 - DNA, 19 bp, CNAG_07724 Southern blot probe primer
gcttcggaggagttgatag

SEQ ID NO: 747 - DNA, 24 bp, NAT#205 STM primer
tatccccctctccgctctctagca

SEQ ID NO: 748 - DNA, 24 bp, STM common primer
gcatgccctgcccctaagaattcg

SEQ ID NO: 749 - DNA, 19 bp, CNAG_06751 5 flanking region primer 1
aaaaacggctgaaggctcg

SEQ ID NO: 750 - DNA, 40 bp, CNAG_06751 5 flanking region primer 2
gctcactggccgtcgttttactggcgagttggtatctgag

SEQ ID NO: 751 - DNA, 40 bp, CNAG_06751 3 flanking region primer 1
catggtcatagctgtttcctgaagatgagagagaaggggg

SEQ ID NO: 752 - DNA, 20 bp, CNAG_06751 3 flanking region primer 2
agaagtggtatgaccgtttg

SEQ ID NO: 753 - DNA, 19 bp, CNAG_06751 diagnostic screening primer, pairing with B79
tccatacattgttgagggc

SEQ ID NO: 754 - DNA, 18 bp, CNAG_06751 Southern blot probe primer
attgcccaagcggataag

SEQ ID NO: 755 - DNA, 22 bp, NAT#208 STM primer
tggtcgcgggagatcgtggttt

SEQ ID NO: 756 - DNA, 24 bp, STM common primer
gcatgccctgcccctaagaattcg

SEQ ID NO: 757 - DNA, 18 bp, CNAG_01438 5 flanking region primer 1
atcacacgcaatcccatc

SEQ ID NO: 758 - DNA, 39 bp, CNAG_01438 5 flanking region primer 2
gctcactggccgtcgttttacagcaagatggaaggaagc

SEQ ID NO: 759 - DNA, 39 bp, CNAG_01438 3 flanking region primer 1
catggtcatagctgtttcctggcgacgaaatcataaggc

SEQ ID NO: 760 - DNA, 19 bp, CNAG_01438 3 flanking region primer 2
tgagaactggacgaactgc

SEQ ID NO: 761 - DNA, 18 bp, CNAG_01438 diagnostic screening primer, pairing with B79
aatgatgcgtcggacttc

SEQ ID NO: 762 - DNA, 20 bp, CNAG_01438 Southern blot probe primer
ggaagagaaagacttgcgag

SEQ ID NO: 763 - DNA, 24 bp, NAT#122 STM primer
acagctccaaacctcgctaaacag

SEQ ID NO: 764 - DNA, 24 bp, STM common primer
gcatgccctgcccctaagaattcg

SEQ ID NO: 765 - DNA, 20 bp, CNAG_00791 5 flanking region primer 1
gcatccattttatcggttcg

SEQ ID NO: 766 - DNA, 41 bp, CNAG_00791 5 flanking region primer 2
gctcactggccgtcgttttacttctgcttgaaggagtcggg

SEQ ID NO: 767 - DNA, 40 bp, CNAG_00791 3 flanking region primer 1
catggtcatagctgtttcctgcggttatcttgcgtaaagc

SEQ ID NO: 768 - DNA, 19 bp, CNAG_00791 3 flanking region primer 2
tgtctcacccatcacgaac

SEQ ID NO: 769 - DNA, 18 bp, CNAG_00791 diagnostic screening primer, pairing with B79
attcgctcaggcagtttc

SEQ ID NO: 770 - DNA, 19 bp, CNAG_00791 Southern blot probe primer
gcgatgatgaggactcttg

SEQ ID NO: 771 - DNA, 21 bp, NAT#146 STM primer
actagccccccctcaccacct

SEQ ID NO: 772 - DNA, 24 bp, STM common primer
gcatgccctgcccctaagaattcg

SEQ ID NO: 773 - DNA, 19 bp, CNAG_02241 5 flanking region primer 1
atagcaaacccatacctcg

SEQ ID NO: 774 - DNA, 37 bp, CNAG_02241 5 flanking region primer 2
tcactggccgtcgttttactttgtttggtagtggggg

SEQ ID NO: 775 - DNA, 40 bp, CNAG_02241 3 flanking region primer 1
catggtcatagctgtttcctgcgagaactctggagcattc

SEQ ID NO: 776 - DNA, 21 bp, CNAG_02241 3 flanking region primer 2
gatgtgttgtggactgtatgc

SEQ ID NO: 777 - DNA, 20 bp, CNAG_02241 diagnostic screening primer, pairing with B79
tcccatcataggagtggacg

SEQ ID NO: 778 - DNA, 20 bp, CNAG_02241 Southern blot probe primer
cttgggagcaaataagtgtg

SEQ ID NO: 779 - DNA, 20 bp, NAT#219 STM primer
ccctaaaaccctacagcaat

SEQ ID NO: 780 - DNA, 24 bp, STM common primer
gcatgccctgcccctaagaattcg

SEQ ID NO: 781 - DNA, 19 bp, CNAG_02566 5 flanking region primer 1
tcgcacggcataggattag

SEQ ID NO: 782 - DNA, 38 bp, CNAG_02566 5 flanking region primer 2
tcactggccgtcgttttacatgccgccagaatgttgag

SEQ ID NO: 783 - DNA, 40 bp, CNAG_02566 3 flanking region primer 1
catggtcatagctgtttcctgtgatgttgatggagactgg

SEQ ID NO: 784 - DNA, 20 bp, CNAG_02566 3 flanking region primer 2
actgcttcttcaccctccac

SEQ ID NO: 785 - DNA, 18 bp, CNAG_02566 diagnostic screening primer, pairing with B79
atctgccgcaacattcac

SEQ ID NO: 786 - DNA, 21 bp, CNAG_02566 Southern blot probe primer
gttggtgcttcatagtgactg

SEQ ID NO: 787 - DNA, 20 bp, NAT#219 STM primer
ccctaaaaccctacagcaat

SEQ ID NO: 788 - DNA, 24 bp, STM common primer
gcatgccctgcccctaagaattcg

SEQ ID NO: 789 - DNA, 19 bp, CNAG_01626 5 flanking region primer 1
ggatgatggaatcgtatgc

SEQ ID NO: 790 - DNA, 38 bp, CNAG_01626 5 flanking region primer 2
tcactggccgtcgttttacattatccaccctcggcttc

SEQ ID NO: 791 - DNA, 42 bp, CNAG_01626 3 flanking region primer 1
catggtcatagctgtttcctggcgaacggtatgacaactatg

SEQ ID NO: 792 - DNA, 22 bp, CNAG_01626 3 flanking region primer 2
ggacgaaaacattgctctcaac

SEQ ID NO: 793 - DNA, 19 bp, CNAG_01626 diagnostic screening primer, pairing with B79
tcagcagcagcaggtaaac

SEQ ID NO: 794 - DNA, 18 bp, CNAG_01626 Southern blot probe primer
cccagaccgttttgaatg

SEQ ID NO: 795 - DNA, 18 bp, NAT#232 STM primer
ctttaaaggtggtttgtg

SEQ ID NO: 796 - DNA, 24 bp, STM common primer
gcatgccctgcccctaagaattcg

SEQ ID NO: 797 - DNA, 20 bp, CNAG_05940 5 flanking region primer 1
tcttgaccgtcgccagttac

SEQ ID NO: 798 - DNA, 39 bp, CNAG_05940 5 flanking region primer 2
tcactggccgtcgttttactggctcaaaggcaaagtcgg

SEQ ID NO: 799 - DNA, 40 bp, CNAG_05940 3 flanking region primer 1
catggtcatagctgtttcctgaggtgattttgggagtcag

SEQ ID NO: 800 - DNA, 19 bp, CNAG_05940 3 flanking region primer 2
ggctgagaatgatgtgacg

SEQ ID NO: 801 - DNA, 19 bp, CNAG_05940 diagnostic screening primer, pairing with B79
ggaaagaagacggatagcg

SEQ ID NO: 802 - DNA, 19 bp, CNAG_05940 Southern blot probe primer
gtctccaggaaagttcgtg

SEQ ID NO: 803 - DNA, 18 bp, NAT#232 STM primer
ctttaaaggtggtttgtg

SEQ ID NO: 804 - DNA, 24 bp, STM common primer
gcatgccctgcccctaagaattcg

SEQ ID NO: 805 - DNA, 22 bp, CNAG_04352 5 flanking region primer 1
gtgattatgtgaacccgttacc

SEQ ID NO: 806 - DNA, 39 bp, CNAG_04352 5 flanking region primer 2
tcactggccgtcgttttacttttagaggtgatgactgcg

SEQ ID NO: 807 - DNA, 41 bp, CNAG_04352 3 flanking region primer 1
catggtcatagctgtttcctgtgctgctggaggaagagaac

SEQ ID NO: 808 - DNA, 19 bp, CNAG_04352 3 flanking region primer 2
agtgagtcgttgatgtggc

SEQ ID NO: 809 - DNA, 19 bp, CNAG_04352 diagnostic screening primer, pairing with B79
atagtgaatacgggtcggg

SEQ ID NO: 810 - DNA, 19 bp, CNAG_04352 Southern blot probe primer
gctgaaacaggaggcatag

SEQ ID NO: 811 - DNA, 20 bp, NAT#234 STM primer
ccagccagcactccgatata

SEQ ID NO: 812 - DNA, 24 bp, STM common primer
gcatgccctgcccctaagaattcg

SEQ ID NO: 813 - DNA, 18 bp, CNAG_03768 5 flanking region primer 1
aatgtccttgcggttgac

SEQ ID NO: 814 - DNA, 40 bp, CNAG_03768 5 flanking region primer 2
gctcactggccgtcgttttacaatagtccccgtcgttgtc

SEQ ID NO: 815 - DNA, 41 bp, CNAG_03768 3 flanking region primer 1
catggtcatagctgtttcctgcgatggatgtttggtggtag

SEQ ID NO: 816 - DNA, 19 bp, CNAG_03768 3 flanking region primer 2
aaaggggttttggtggctc

SEQ ID NO: 817 - DNA, 20 bp, CNAG_03768 diagnostic screening primer, pairing with B79
tggatttggcagagaagaag

SEQ ID NO: 818 - DNA, 19 bp, CNAG_03768 Southern blot probe primer
aagacacttggctctccag

SEQ ID NO: 819 - DNA, 20 bp, NAT#234 STM primer
ccagccagcactccgatata

SEQ ID NO: 820 - DNA, 24 bp, STM common primer
gcatgccctgcccctaagaattcg

SEQ ID NO: 821 - DNA, 20 bp, CNAG_02322 5 flanking region primer 1
cgctcactcacctttcaaac

SEQ ID NO: 822 - DNA, 35 bp, CNAG_02322 5 flanking region primer 2
ctggccgtcgttttacacatcggcttttacggagc

SEQ ID NO: 823 - DNA, 37 bp, CNAG_02322 3 flanking region primer 1
gtcatagctgtttcctgctcggttaccagtcactacg

SEQ ID NO: 824 - DNA, 20 bp, CNAG_02322 3 flanking region primer 2
ccaccaagattcagagttcg

SEQ ID NO: 825 - DNA, 19 bp, CNAG_02322 diagnostic screening primer, pairing with B79
gagatttcggtggatttcc

SEQ ID NO: 826 - DNA, 18 bp, CNAG_02322 Southern blot probe primer
aagcaaccctcagcattg

SEQ ID NO: 827 - DNA, 20 bp, NAT#240 STM primer
ggtgttggatcggggtggat

SEQ ID NO: 828 - DNA, 24 bp, STM common primer
gcatgccctgcccctaagaattcg

SEQ ID NO: 829 - DNA, 20 bp, CNAG_06818 5 flanking region primer 1
tgtattctgcccacctccac

SEQ ID NO: 830 - DNA, 39 bp, CNAG_06818 5 flanking region primer 2
tcactggccgtcgttttaccctctttgctggtctctgag

SEQ ID NO: 831 - DNA, 41 bp, CNAG_06818 3 flanking region primer 1
catggtcatagctgtttcctgtctgctgctacatcaggttc

SEQ ID NO: 832 - DNA, 19 bp, CNAG_06818 3 flanking region primer 2
aacctctgtatcgctgacg

SEQ ID NO: 833 - DNA, 22 bp, CNAG_06818 diagnostic screening primer, pairing with B79
gggtgaaagacaataggtaagg

SEQ ID NO: 834 - DNA, 21 bp, CNAG_06818 Southern blot probe primer
aaagtgaagagaggaggtcag

SEQ ID NO: 835 - DNA, 20 bp, NAT#240 STM primer
ggtgttggatcggggtggat

SEQ ID NO: 836 - DNA, 24 bp, STM common primer
gcatgccctgcccctaagaattcg

SEQ ID NO: 837 - DNA, 19 bp, CNAG_07011 5 flanking region primer 1
ccaacaaatagcaaagccg

SEQ ID NO: 838 - DNA, 38 bp, CNAG_07011 5 flanking region primer 2
tcactggccgtcgttttacacaccaaagccaagaacac

SEQ ID NO: 839 - DNA, 41 bp, CNAG_07011 3 flanking region primer 1
catggtcatagctgtttcctggctaatgcctgaaacagacc

SEQ ID NO: 840 - DNA, 19 bp, CNAG_07011 3 flanking region primer 2
tcggacacccaatcaatac

SEQ ID NO: 841 - DNA, 18 bp, CNAG_07011 diagnostic screening primer, pairing with B79
ttgtgttgttcggtgagg

SEQ ID NO: 842 - DNA, 20 bp, CNAG_07011 Southern blot probe primer
tgggtgatacagaggaaaac

SEQ ID NO: 843 - DNA, 24 bp, NAT#273 STM primer
gagatctttcgggaggtctggatt

SEQ ID NO: 844 - DNA, 24 bp, STM common primer
gcatgccctgcccctaagaattcg

SEQ ID NO: 845 - DNA, 20 bp, CNAG_04036 5 flanking region primer 1
ccagttgaacgcttctaaac

SEQ ID NO: 846 - DNA, 39 bp, CNAG_04036 5 flanking region primer 2
tcactggccgtcgttttactgatggtgtgggaacaatac

SEQ ID NO: 847 - DNA, 40 bp, CNAG_04036 3 flanking region primer 1
catggtcatagctgtttcctgttctccttgcctatgtgcc

SEQ ID NO: 848 - DNA, 20 bp, CNAG_04036 3 flanking region primer 2
cagcaacttactttggaggc

SEQ ID NO: 849 - DNA, 19 bp, CNAG_04036 diagnostic screening primer, pairing with B79
atagacagcagcgggatac

SEQ ID NO: 850 - DNA, 18 bp, CNAG_04036 Southern blot probe primer
tcacagatgcctttctcg

SEQ ID NO: 851 - DNA, 24 bp, NAT#273 STM primer
gagatctttcgggaggtctggatt

SEQ ID NO: 852 - DNA, 24 bp, STM common primer
gcatgccctgcccctaagaattcg

SEQ ID NO: 853 - DNA, 19 bp, CNAG_07506 5 flanking region primer 1
cgtaatgacactggagagc

SEQ ID NO: 854 - DNA, 42 bp, CNAG_07506 5 flanking region primer 2
gctcactggccgtcgttttactgttgccgtaggaaccgcttc

SEQ ID NO: 855 - DNA, 40 bp, CNAG_07506 3 flanking region primer 1
catggtcatagctgtttcctgtcccaaagcctcttctcag

SEQ ID NO: 856 - DNA, 18 bp, CNAG_07506 3 flanking region primer 2
gtgagaccctgatagacc

SEQ ID NO: 857 - DNA, 19 bp, CNAG_07506 diagnostic screening primer, pairing with B79
gactcaaagggagatgacg

SEQ ID NO: 858 - DNA, 19 bp, CNAG_07506 Southern blot probe primer
gcttttgcctgctattgac

SEQ ID NO: 859 - DNA, 20 bp, NAT#296 STM primer
cgcccgccctcactatccac

SEQ ID NO: 860 - DNA, 24 bp, STM common primer
gcatgccctgcccctaagaattcg

SEQ ID NO: 861 - DNA, 19 bp, CNAG_06223 5 flanking region primer 1
ggatgaaggggaagacttg

SEQ ID NO: 862 - DNA, 38 bp, CNAG_06223 5 flanking region primer 2
tcactggccgtcgttttaccttccgttcaaaatcgtcg

SEQ ID NO: 863 - DNA, 41 bp, CNAG_06223 3 flanking region primer 1
catggtcatagctgtttcctggtctaccaccaccatcacac

SEQ ID NO: 864 - DNA, 20 bp, CNAG_06223 3 flanking region primer 2
gccgtccattcatacatctg

SEQ ID NO: 865 - DNA, 19 bp, CNAG_06223 diagnostic screening primer, pairing with B79
ggtgtcaatagttgggtgg

SEQ ID NO: 866 - DNA, 19 bp, CNAG_06223 Southern blot probe primer
agagcagaagcaaatgacc

SEQ ID NO: 867 - DNA, 20 bp, NAT#210 STM primer
ctagagcccgccacaacgct

SEQ ID NO: 868 - DNA, 24 bp, STM common primer
gcatgccctgcccctaagaattcg

SEQ ID NO: 869 - DNA, 24 bp, CNAG_06283 5 flanking region primer 1
ccctttgtccttacccacattttc

SEQ ID NO: 870 - DNA, 39 bp, CNAG_06283 5 flanking region primer 2
tcactggccgtcgttttactcgttcgggcacttcttgac

SEQ ID NO: 871 - DNA, 41 bp, CNAG_06283 3 flanking region primer 1
catggtcatagctgtttcctgcgagtaaggagacggttgag

SEQ ID NO: 872 - DNA, 22 bp, CNAG_06283 3 flanking region primer 2
ggttagggggataaaataggag

SEQ ID NO: 873 - DNA, 21 bp, CNAG_06283 diagnostic screening primer, pairing with B79
gagacattctttctgacgagc

SEQ ID NO: 874 - DNA, 20 bp, CNAG_06283 Southern blot probe primer
tggcttgaagggtcttggtc

SEQ ID NO: 875 - DNA, 20 bp, NAT#234 STM primer
ccagccagcactccgatata

SEQ ID NO: 876 - DNA, 24 bp, STM common primer
gcatgccctgcccctaagaattcg

SEQ ID NO: 877 - DNA, 22 bp, CNAG_04583 5 flanking region primer 1
gctcgctacattttcaggtatc

SEQ ID NO: 878 - DNA, 39 bp, CNAG_04583 5 flanking region primer 2
tcactggccgtcgttttacgagagggtcggaaatagaag

SEQ ID NO: 879 - DNA, 41 bp, CNAG_04583 3 flanking region primer 1
catggtcatagctgtttcctggggaaggagtaatgcctgac

SEQ ID NO: 880 - DNA, 18 bp, CNAG_04583 3 flanking region primer 2
aaccgtgatggagattgg

SEQ ID NO: 881 - DNA, 20 bp, CNAG_04583 diagnostic screening primer, pairing with B79
cggtgtgcgattctaacttc

SEQ ID NO: 882 - DNA, 19 bp, CNAG_04583 Southern blot probe primer
ggggactgttttgatgacc

SEQ ID NO: 883 - DNA, 24 bp, NAT#102 STM primer
ccatagcgatatctaccccaatct

SEQ ID NO: 884 - DNA, 24 bp, STM common primer
gcatgccctgcccctaagaattcg

SEQ ID NO: 885 - DNA, 19 bp, CNAG_03261 5 flanking region primer 1
ggcgataaagacgacgaac

SEQ ID NO: 886 - DNA, 35 bp, CNAG_03261 5 flanking region primer 2
ctggccgtcgttttacggactattcgtggcttagc

SEQ ID NO: 887 - DNA, 35 bp, CNAG_03261 3 flanking region primer 1
gtcatagctgtttcctgtgagaccaatgtgttgcc

SEQ ID NO: 888 - DNA, 24 bp, CNAG_03261 3 flanking region primer 2
cctcaacccctttctgatttatcc

SEQ ID NO: 889 - DNA, 22 bp, CNAG_03261 diagnostic screening primer, pairing with B79
tagtcggtgatgagagttgcgg

SEQ ID NO: 890 - DNA, 20 bp, CNAG_03261 Southern blot probe primer
gcaaatctgcttctgggatg

SEQ ID NO: 891 - DNA, 19 bp, CNAG_04908 5 flanking region primer 1
gatgacgaatagcacggtc

SEQ ID NO: 892 - DNA, 37 bp, CNAG_04908 5 flanking region primer 2
tcactggccgtcgttttacggatgggaagattgttgg

SEQ ID NO: 893 - DNA, 39 bp, CNAG_04908 3 flanking region primer 1
gatggtcatagctgtttcctgttgcttacgcctttgtcc

SEQ ID NO: 894 - DNA, 18 bp, CNAG_04908 3 flanking region primer 2
atggttgttcacgcacag

SEQ ID NO: 895 - DNA, 18 bp, CNAG_04908 diagnostic screening primer, pairing with B79
aaacaaaagccgagggag

SEQ ID NO: 896 - DNA, 19 bp, CNAG_04908 Southern blot probe primer
aacttcccaccccttcatc

SEQ ID NO: 897 - DNA, 24 bp, NAT#242 STM primer
gtagcgataggggtgtcgctttag

SEQ ID NO: 898 - DNA, 24 bp, STM common primer
gcatgccctgcccctaagaattcg

SEQ ID NO: 899 - DNA, 19 bp, CNAG_01317 5 flanking region primer 1
aagcaccaagaagcaagtg

SEQ ID NO: 900 - DNA, 37 bp, CNAG_01317 5 flanking region primer 2
tcactggccgtcgttttacattgacacctgccgattc

SEQ ID NO: 901 - DNA, 40 bp, CNAG_01317 3 flanking region primer 1
catggtcatagctgtttcctgtactatcagcagaagcggc

SEQ ID NO: 902 - DNA, 20 bp, CNAG_01317 3 flanking region primer 2
aatgataggcggaagtaagg

SEQ ID NO: 903 - DNA, 19 bp, CNAG_01317 diagnostic screening primer, pairing with B79
ccacctcgcagtatcaaac

SEQ ID NO: 904 - DNA, 20 bp, CNAG_01317 Southern blot probe primer
agggtcagggagatgatgtg

SEQ ID NO: 905 - DNA, 19 bp, CNAG_00559 5 flanking region primer 1
ggtgtttccatacgaaccg

SEQ ID NO: 906 - DNA, 38 bp, CNAG_00559 5 flanking region primer 2; identical to SEQ ID NO: 701

SEQ ID NO: 907 - DNA, 35 bp, CNAG_00559 3 flanking region primer 1; identical to SEQ ID NO: 702

SEQ ID NO: 908 - DNA, 20 bp, CNAG_00559 3 flanking region primer 2
gctgagaaggagaggatagc

SEQ ID NO: 909 - DNA, 20 bp, CNAG_00559 diagnostic screening primer, pairing with B79
gtggttgaaagtattaggcg

SEQ ID NO: 910 - DNA, 19 bp, CNAG_00559 Southern blot probe primer
tctcttcgtttgctacacg

SEQ ID NO: 911 - DNA, 24 bp, NAT#242 STM primer
gtagcgataggggtgtcgctttag

SEQ ID NO: 912 - DNA, 24 bp, STM common primer
gcatgccctgcccctaagaattcg

SEQ ID NO: 913 - DNA, 18 bp, CNAG_07940 5 flanking region primer 1
caaggtaatgattggggc

SEQ ID NO: 914 - DNA, 38 bp, CNAG_07940 5 flanking region primer 2
tcactggccgtcgttttacgcaataatggaaggtctcg

SEQ ID NO: 915 - DNA, 39 bp, CNAG_07940 3 flanking region primer 1
catggtcatagctgtttcctgatcaagaatgacacgccg

SEQ ID NO: 916 - DNA, 19 bp, CNAG_07940 3 flanking region primer 2
aacttgtatggtggtgccg

SEQ ID NO: 917 - DNA, 19 bp, CNAG_07940 diagnostic screening primer, pairing with B79
tcacttgctcttctccctg

SEQ ID NO: 918 - DNA, 18 bp, CNAG_07940 Southern blot probe primer
gtgacgaatgcgaaactc

SEQ ID NO: 919 - DNA, 20 bp, NAT#191 STM primer
atatggatgtttttagcgag

SEQ ID NO: 920 - DNA, 24 bp, STM common primer
gcatgccctgcccctaagaattcg

SEQ ID NO: 921 - DNA, 18 bp, CNAG_05535 5 flanking region primer 1
agcaacaacggcatagtg

SEQ ID NO: 922 - DNA, 39 bp, CNAG_05535 5 flanking region primer 2
tcactggccgtcgttttacacgacagtgagagtcctgac

SEQ ID NO: 923 - DNA, 43 bp, CNAG_05535 3 flanking region primer 1
catggtcatagctgtttcctgctggagcgaggaaatagtaatg

SEQ ID NO: 924 - DNA, 18 bp, CNAG_05535 3 flanking region primer 2
acacaaagcgagtggttg

SEQ ID NO: 925 - DNA, 19 bp, CNAG_05535 diagnostic screening primer, pairing with B79
ggcagtgtcagatgaaagc

SEQ ID NO: 926 - DNA, 19 bp, CNAG_05535 Southern blot probe primer
catcggctacatcttcctc

SEQ ID NO: 927 - DNA, 21 bp, CNAG_02516 5 flanking region primer 1
gcatcacacgaacgattctac

SEQ ID NO: 928 - DNA, 38 bp, CNAG_02516 5 flanking region primer 2
tcactggccgtcgttttacattgttggcggtggaaacg

SEQ ID NO: 929 - DNA, 41 bp, CNAG_02516 3 flanking region primer 1
catggtcatagctgtttcctgaggtttgggagcagtaaggc

SEQ ID NO: 930 - DNA, 19 bp, CNAG_02516 3 flanking region primer 2
gatgtttgtgaccgattcg

SEQ ID NO: 931 - DNA, 19 bp, CNAG_02516 diagnostic screening primer, pairing with B79
gcgaaggtttaccgataag

SEQ ID NO: 932 - DNA, 20 bp, CNAG_02516 Southern blot probe primer
tatggggttaggagcgttgg

SEQ ID NO: 933 - DNA, 20 bp, NAT#210 STM primer
ctagagcccgccacaacgct

SEQ ID NO: 934 - DNA, 24 bp, STM common primer
gcatgccctgcccctaagaattcg

SEQ ID NO: 935 - DNA, 19 bp, CNAG_04226 5 flanking region primer 1
gccctttttggtatgacag

SEQ ID NO: 936 - DNA, 38 bp, CNAG_04226 5 flanking region primer 2
tcactggccgtcgttttactgtgagggattccttgttc

SEQ ID NO: 937 - DNA, 39 bp, CNAG_04226 3 flanking region primer 1
catggtcatagctgtttcctggttggaaacaagcagtcg

SEQ ID NO: 938 - DNA, 20 bp, CNAG_04226 3 flanking region primer 2
tcagaagaatcaagaggtcg

SEQ ID NO: 939 - DNA, 19 bp, CNAG_04226 diagnostic screening primer, pairing with B79
acttacattgccttcctcg

SEQ ID NO: 940 - DNA, 19 bp, CNAG_04226 Southern blot probe primer
atacatcagcctgtcctgc

SEQ ID NO: 941 - DNA, 19 bp, CNAG_05170 5 flanking region primer 1
tgccttcgctctgtaactc

SEQ ID NO: 942 - DNA, 34 bp, CNAG_05170 5 flanking region primer 2
ctggccgtcgttttaccctttttgaggctcgctg

SEQ ID NO: 943 - DNA, 36 bp, CNAG_05170 3 flanking region primer 1
gtcatagctgtttcctgaaatgaaggagtgtgcggg

SEQ ID NO: 944 - DNA, 20 bp, CNAG_05170 3 flanking region primer 2
aataggacctcaacaccagg

SEQ ID NO: 945 - DNA, 18 bp, CNAG_05170 diagnostic screening primer, pairing with B79
aacaagaagcccctttcg

SEQ ID NO: 946 - DNA, 18 bp, CNAG_05170 Southern blot probe primer
agtttttggacccgagtg

SEQ ID NO: 947 - DNA, 18 bp, NAT#232 STM primer
ctttaaaggtggtttgtg

SEQ ID NO: 948 - DNA, 24 bp, STM common primer
gcatgccctgcccctaagaattcg

SEQ ID NO: 949 - DNA, 20 bp, CNAG_03902 5 flanking region primer 1
gcaaagtcaagaaggtcagg

SEQ ID NO: 950 - DNA, 35 bp, CNAG_03902 5 flanking region primer 2
ctggccgtcgttttacttcttctttggctcgtccg

SEQ ID NO: 951 - DNA, 39 bp, CNAG_03902 3 flanking region primer 1
gtcatagctgtttcctggggagatgaaatgtgcgtttag

SEQ ID NO: 952 - DNA, 22 bp, CNAG_03902 3 flanking region primer 2
atgctttcgccgtcatctcgtc

SEQ ID NO: 953 - DNA, 20 bp, CNAG_03902 diagnostic screening primer, pairing with B79
tgattacccctgtcaaactc

SEQ ID NO: 954 - DNA, 19 bp, CNAG_03902 Southern blot probe primer
cagaatcgggaagtaatgg

SEQ ID NO: 955 - DNA, 18 bp, NAT#232 STM primer
ctttaaaggtggtttgtg

SEQ ID NO: 956 - DNA, 24 bp, STM common primer
gcatgccctgcccctaagaattcg

SEQ ID NO: 957 - DNA, 20 bp, CNAG_06097 5 flanking region primer 1
cagtccgaagtttacaatcg

SEQ ID NO: 958 - DNA, 36 bp, CNAG_06097 5 flanking region primer 2
ctggccgtcgttttactttcgtcgtgtggagttggc

SEQ ID NO: 959 - DNA, 37 bp, CNAG_06097 3 flanking region primer 1
gtcatagctgtttcctgagattggagggtttgagggc

SEQ ID NO: 960 - DNA, 19 bp, CNAG_06097 3 flanking region primer 2
tccaccgaagaaactgaag

SEQ ID NO: 961 - DNA, 20 bp, CNAG_06097 diagnostic screening primer, pairing with B79
aggtttgagaggtttggaag

SEQ ID NO: 962 - DNA, 18 bp, CNAG_06097 Southern blot probe primer
attatcggagcgttgtgg

SEQ ID NO: 963 - DNA, 20 bp, CNAG_03431 5 flanking region primer 1
aagcactctgtagcctgttg

SEQ ID NO: 964 - DNA, 39 bp, CNAG_03431 5 flanking region primer 2
gctcactggccgtcgttttaccttgaagatgatgcgtgc

SEQ ID NO: 965 - DNA, 40 bp, CNAG_03431 3 flanking region primer 1
catggtcatagctgtttcctgcgctcatagagaatgctgg

SEQ ID NO: 966 - DNA, 19 bp, CNAG_03431 3 flanking region primer 2
taggagtgtctgccaaagc

SEQ ID NO: 967 - DNA, 19 bp, CNAG_03431 diagnostic screening primer, pairing with B79
tcatcctcatcccgaatac

SEQ ID NO: 968 - DNA, 19 bp, CNAG_03431 Southern blot probe primer
actcttcgtgagacgcatc

SEQ ID NO: 969 - DNA, 24 bp, NAT#290 STM primer
accgacagctcgaacaagcaagag

SEQ ID NO: 970 - DNA, 24 bp, STM common primer
gcatgccctgcccctaagaattcg

SEQ ID NO: 971 - DNA, 21 bp, CNAG_00830 5 flanking region primer 1
ccgactaataggtgtgctgtc

SEQ ID NO: 972 - DNA, 41 bp, CNAG_00830 5 flanking region primer 2
gctcactggccgtcgttttacgagatgagatgagttgcgtg

SEQ ID NO: 973 - DNA, 41 bp, CNAG_00830 3 flanking region primer 1
catggtcatagctgtttcctgttgtgtccccatcactaccg

SEQ ID NO: 974 - DNA, 19 bp, CNAG_00830 3 flanking region primer 2
catccaaagaagcgaaacg

SEQ ID NO: 975 - DNA, 24 bp, CNAG_00830 diagnostic screening primer, pairing with B79
gaagagaagtagtggatagactcg

SEQ ID NO: 976 - DNA, 19 bp, CNAG_00830 Southern blot probe primer
tgatgccgtaaatcgtagg

SEQ ID NO: 977 - DNA, 21 bp, NAT#292 STM primer
atttcgatgtatatatgtagc

SEQ ID NO: 978 - DNA, 24 bp, STM common primer
gcatgccctgcccctaagaattcg

SEQ ID NO: 979 - DNA, 20 bp, CNAG_07443 5 flanking region primer 1
atctcttctctcggcgtgtc

SEQ ID NO: 980 - DNA, 40 bp, CNAG_07443 5 flanking region primer 2
gctcactggccgtcgttttacacaggaaaaggaggagtcg

SEQ ID NO: 981 - DNA, 40 bp, CNAG_07443 3 flanking region primer 1
catggtcatagctgtttcctgaagtctttccgtctgaccc

SEQ ID NO: 982 - DNA, 18 bp, CNAG_07443 3 flanking region primer 2
tcgcatcccttgtattcg

SEQ ID NO: 983 - DNA, 19 bp, CNAG_07443 diagnostic screening primer, pairing with B79
tcaataatcagccgcctac

SEQ ID NO: 984 - DNA, 19 bp, CNAG_07443 Southern blot probe primer
ttagattccgcataggtcc

SEQ ID NO: 985 - DNA, 21 bp, NAT#295 STM primer
acacctacatcaaaccctccc

SEQ ID NO: 986 - DNA, 24 bp, STM common primer
gcatgccctgcccctaagaattcg

SEQ ID NO: 987 - DNA, 19 bp, CNAG_05186 5 flanking region primer 1
acaacggtcaagaagggtc

SEQ ID NO: 988 - DNA, 39 bp, CNAG_05186 5 flanking region primer 2
gctcactggccgtcgttttacaagtaaaggaacgcacgg

SEQ ID NO: 989 - DNA, 41 bp, CNAG_05186 3 flanking region primer 1
catggtcatagctgtttcctgcgcttgagacgggagtaatc

SEQ ID NO: 990 - DNA, 20 bp, CNAG_05186 3 flanking region primer 2
gaggtaaggatgattggacc

SEQ ID NO: 991 - DNA, 23 bp, CNAG_05186 diagnostic screening primer, pairing with B79
gtgtgaagtgagtagtaacgagc

SEQ ID NO: 992 - DNA, 22 bp, CNAG_05186 Southern blot probe primer
ttccctatctctcttcataccc

SEQ ID NO: 993 - DNA, 20 bp, NAT#296 STM primer
cgcccgccctcactatccac

SEQ ID NO: 994 - DNA, 24 bp, STM common primer
gcatgccctgcccctaagaattcg

SEQ ID NO: 995 - DNA, 20 bp, CNAG_03561 5 flanking region primer 1
tgggcgagacgagatagaac

SEQ ID NO: 996 - DNA, 36 bp, CNAG_03561 5 flanking region primer 2
ctggccgtcgttttacggataaagatgattcgggtc

SEQ ID NO: 997 - DNA, 36 bp, CNAG_03561 3 flanking region primer 1
gtcatagctgtttcctgtgatggctgatttcccgtg

SEQ ID NO: 998 - DNA, 36 bp, CNAG_03561 3 flanking region primer 2; identical to SEQ ID NO: 997

SEQ ID NO: 999 - DNA, 20 bp, CNAG_03561 diagnostic screening primer, pairing with B79
aagaaagacggtagcggtgg

SEQ ID NO: 1000 - DNA, 20 bp, CNAG_03561 Southern blot probe primer
ccacctcttcatccaatagc

SEQ ID NO: 1001 - DNA, 20 bp, NAT#43 STM primer
ccagctaccaatcacgctac

SEQ ID NO: 1002 - DNA, 24 bp, STM common primer
gcatgccctgcccctaagaattcg

SEQ ID NO: 1003 - DNA, 19 bp, CNAG_04878 5 flanking region primer 1
aagtccgtgctggctaatc

SEQ ID NO: 1004 - DNA, 35 bp, CNAG_04878 5 flanking region primer 2
ctggccgtcgttttaccttttcgctgccttattcg

SEQ ID NO: 1005 - DNA, 41 bp, CNAG_04878 3 flanking region primer 1
gtcatagctgtttcctgaaaacagggcatacggtgtcgtgg

SEQ ID NO: 1006 - DNA, 20 bp, CNAG_04878 3 flanking region primer 2
gctgaccatctcttccctac

SEQ ID NO: 1007 - DNA, 22 bp, CNAG_04878 diagnostic screening primer, pairing with B79
ccttgtttgtgtctaccgtatc

SEQ ID NO: 1008 - DNA, 19 bp, CNAG_04878 Southern blot probe primer
agtgggaatcgtcgttgac

SEQ ID NO: 1009 - DNA, 20 bp, NAT#116 STM primer
gcacccaagagctccatctc

SEQ ID NO: 1010 - DNA, 24 bp, STM common primer
gcatgccctgcccctaagaattcg

SEQ ID NO: 1011 - DNA, 19 bp, CNAG_03279 5 flanking region primer 1
cgtttccagttatcgcttc

SEQ ID NO: 1012 - DNA, 41 bp, CNAG_03279 5 flanking region primer 2
gctcactggccgtcgttttacgcaatgacccactttttgac

SEQ ID NO: 1013 - DNA, 41 bp, CNAG_03279 3 flanking region primer 1
catggtcatagctgtttcctggctttgcctgatgagttttg

SEQ ID NO: 1014 - DNA, 19 bp, CNAG_03279 3 flanking region primer 2
gtaacccactcggaagttg

SEQ ID NO: 1015 - DNA, 19 bp, CNAG_03279 diagnostic screening primer, pairing with B79
ttgtctgtgaggtggaagg

SEQ ID NO: 1016 - DNA, 20 bp, CNAG_03279 Southern blot probe primer
caggctcgtttgtagccttc

SEQ ID NO: 1017 - DNA, 24 bp, NAT#122 STM primer
acagctccaaacctcgctaaacag

SEQ ID NO: 1018 - DNA, 24 bp, STM common primer
gcatgccctgcccctaagaattcg

SEQ ID NO: 1019 - DNA, 18 bp, CNAG_06921 5 flanking region primer 1
gacaaagcaacaacagcg

SEQ ID NO: 1020 - DNA, 37 bp, CNAG_06921 5 flanking region primer 2
tcactggccgtcgttttactcggatgacagatggttg

SEQ ID NO: 1021 - DNA, 39 bp, CNAG_06921 3 flanking region primer 1
catggtcatagctgtttcctgaaagattgggcgtctctg

SEQ ID NO: 1022 - DNA, 18 bp, CNAG_06921 3 flanking region primer 2
atcatcagcgacatccag

SEQ ID NO: 1023 - DNA, 18 bp, CNAG_06921 diagnostic screening primer, pairing with B79
aaagaacatacacgccgc

SEQ ID NO: 1024 - DNA, 18 bp, CNAG_06921 Southern blot probe primer
accatctggatttctgcc

SEQ ID NO: 1025 - DNA, 21 bp, NAT#159 STM primer
acgcaccagacacacaaccag

SEQ ID NO: 1026 - DNA, 24 bp, STM common primer
gcatgccctgcccctaagaattcg

SEQ ID NO: 1027 - DNA, 20 bp, CNAG_02555 5 flanking region primer 1
agaggaacacggtatggtcg

SEQ ID NO: 1028 - DNA, 40 bp, CNAG_02555 5 flanking region primer 2
gctcactggccgtcgttttaccaacaacggtgaaccaaag

SEQ ID NO: 1029 - DNA, 41 bp, CNAG_02555 3 flanking region primer 1
catggtcatagctgtttcctgcagagtggaggtagaaacgg

SEQ ID NO: 1030 - DNA, 18 bp, CNAG_02555 3 flanking region primer 2
tctgaaatgctggctgtc

SEQ ID NO: 1031 - DNA, 20 bp, CNAG_02555 diagnostic screening primer, pairing with B79
cccctcacaacttgctaatg

SEQ ID NO: 1032 - DNA, 20 bp, CNAG_02555 Southern blot probe primer
ccgatgtcgacgtatgattg

SEQ ID NO: 1033 - DNA, 18 bp, NAT#270 STM primer
ggtggtttgtgtgggtag

SEQ ID NO: 1034 - DNA, 24 bp, STM common primer
gcatgccctgcccctaagaattcg

SEQ ID NO: 1035 - DNA, 19 bp, CNAG_03710 5 flanking region primer 1
aagacaagaagcagcagcg

SEQ ID NO: 1036 - DNA, 40 bp, CNAG_03710 5 flanking region primer 2
gctcactggccgtcgttttactatcattcccatccgtcgc

SEQ ID NO: 1037 - DNA, 42 bp, CNAG_03710 3 flanking region primer 1
catggtcatagctgtttcctgcgctcaataacatcgtcagac

SEQ ID NO: 1038 - DNA, 20 bp, CNAG_03710 3 flanking region primer 2
ccagccttcatctctcttcc

SEQ ID NO: 1039 - DNA, 20 bp, CNAG_03710 diagnostic screening primer, pairing with B79
cagaactgataactggctgc

SEQ ID NO: 1040 - DNA, 20 bp, CNAG_03710 Southern blot probe primer
tcctctgcaccaagactgtg

SEQ ID NO: 1041 - DNA, 24 bp, NAT#290 STM primer
accgacagctcgaacaagcaagag

SEQ ID NO: 1042 - DNA, 24 bp, STM common primer
gcatgccctgcccctaagaattcg

SEQ ID NO: 1043 - DNA, 20 bp, CNAG_03183 5 flanking region primer 1
ctctatgagggcaaagtcag

SEQ ID NO: 1044 - DNA, 40 bp, CNAG_03183 5 flanking region primer 2
gctcactggccgtcgttttactgttgttgctgttggctcg

SEQ ID NO: 1045 - DNA, 40 bp, CNAG_03183 3 flanking region primer 1
catggtcatagctgtttcctgttcttccaatcccagccac

SEQ ID NO: 1046 - DNA, 19 bp, CNAG_03183 3 flanking region primer 2
tacgcttcacagattacgc

SEQ ID NO: 1047 - DNA, 18 bp, CNAG_03183 diagnostic screening primer, pairing with B79
tatacgtccaagacatcc

SEQ ID NO: 1048 - DNA, 20 bp, CNAG_03183 Southern blot probe primer
ctgattccgaggcttactcg

SEQ ID NO: 1049 - DNA, 21 bp, NAT#292 STM primer
atttcgatgtatatatgtagc

SEQ ID NO: 1050 - DNA, 24 bp, STM common primer
gcatgccctgcccctaagaattcg

SEQ ID NO: 1051 - DNA, 20 bp, CNAG_04637 5 flanking region primer 1
ccttcaagccaaaatgagac

SEQ ID NO: 1052 - DNA, 40 bp, CNAG_04637 5 flanking region primer 2
gctcactggccgtcgttttacgagatggagagaagcaacg

SEQ ID NO: 1053 - DNA, 43 bp, CNAG_04637 3 flanking region primer 1
catggtcatagctgtttcctgggttgacggatttactgaagtc

SEQ ID NO: 1054 - DNA, 20 bp, CNAG_04637 3 flanking region primer 2
tggaagatgactcactcggg

SEQ ID NO: 1055 - DNA, 19 bp, CNAG_04637 diagnostic screening primer, pairing with B79
tccatcaaagatacacccg

SEQ ID NO: 1056 - DNA, 20 bp, CNAG_04637 Southern blot probe primer
ttacatcttgaggcttagcg

SEQ ID NO: 1057 - DNA, 20 bp, NAT#296 STM primer
cgcccgccctcactatccac

SEQ ID NO: 1058 - DNA, 24 bp, STM common primer
gcatgccctgcccctaagaattcg

SEQ ID NO: 1059 - DNA, 19 bp, CNAG_04398 5 flanking region primer 1
agtctggagaaaaggggtc

SEQ ID NO: 1060 - DNA, 34 bp, CNAG_04398 5 flanking region primer 2
ctggccgtcgttttacgcaaacacacattctcgg

SEQ ID NO: 1061 - DNA, 36 bp, CNAG_04398 3 flanking region primer 1
gtcatagctgtttcctgttggctaatgtagggttgg

SEQ ID NO: 1062 - DNA, 18 bp, CNAG_04398 3 flanking region primer 2
ccccttcccatttttcac

SEQ ID NO: 1063 - DNA, 22 bp, CNAG_04398 diagnostic screening primer, pairing with B79
gccactttctgatttccgtatc

SEQ ID NO: 1064 - DNA, 18 bp, CNAG_04398 Southern blot probe primer
tatttgctgcctgaccac

SEQ ID NO: 1065 - DNA, 20 bp, NAT#225 STM primer
ccatagaactagctaaagca

SEQ ID NO: 1066 - DNA, 24 bp, STM common primer
gcatgccctgcccctaagaattcg

SEQ ID NO: 1067 - DNA, 20 bp, CNAG_01454 5 flanking region primer 1
ggaagtttggaggaggatag

SEQ ID NO: 1068 - DNA, 37 bp, CNAG_01454 5 flanking region primer 2
tcactggccgtcgttttaccagattcgtggtcaaagc

SEQ ID NO: 1069 - DNA, 40 bp, CNAG_01454 3 flanking region primer 1
catggtcatagctgtttcctggccttgaatgatgaccagc

SEQ ID NO: 1070 - DNA, 18 bp, CNAG_01454 3 flanking region primer 2
cggatttgagatgatgcc

SEQ ID NO: 1071 - DNA, 22 bp, CNAG_01454 diagnostic screening primer, pairing with B79
gttagaggagtcattctttggc

SEQ ID NO: 1072 - DNA, 20 bp, CNAG_01454 Southern blot probe primer
caaaaggtcaaggaaaggtg

SEQ ID NO: 1073 - DNA, 24 bp, NAT#58 STM primer
cgcaaaatcactagccctatagcg

SEQ ID NO: 1074 - DNA, 24 bp, STM common primer
gcatgccctgcccctaagaattcg

SEQ ID NO: 1075 - DNA, 18 bp, CNAG_04268 5 flanking region primer 1
tcgtctttgtgtggttgc

SEQ ID NO: 1076 - DNA, 38 bp, CNAG_04268 5 flanking region primer 2
tcactggccgtcgttttacacttatggcgacttacggg

SEQ ID NO: 1077 - DNA, 40 bp, CNAG_04268 3 flanking region primer 1
catggtcatagctgtttcctggcaatgtctgtatcaccgc

SEQ ID NO: 1078 - DNA, 19 bp, CNAG_04268 3 flanking region primer 2
cgtccgcctgtattttatc

SEQ ID NO: 1079 - DNA, 18 bp, CNAG_04268 diagnostic screening primer, pairing with B79
atgatgctgttttgcccc

SEQ ID NO: 1080 - DNA, 18 bp, CNAG_04268 Southern blot probe primer
ttctttccacatcggtcc

SEQ ID NO: 1081 - DNA, 24 bp, NAT#102 STM primer
ccatagcgatatctaccccaatct

SEQ ID NO: 1082 - DNA, 24 bp, STM common primer
gcatgccctgcccctaagaattcg

SEQ ID NO: 1083 - DNA, 22 bp, CNAG_00031 5 flanking region primer 1
atccaatcatcggcttcccagc

SEQ ID NO: 1084 - DNA, 35 bp, CNAG_00031 5 flanking region primer 2
ctggccgtcgttttacacttgaactcccatctgcg

SEQ ID NO: 1085 - DNA, 37 bp, CNAG_00031 3 flanking region primer 1
gtcatagctgtttcctggaaatgcgatgaatgggttg

SEQ ID NO: 1086 - DNA, 21 bp, CNAG_00031 3 flanking region primer 2
cctcttgccctaatgagatag

SEQ ID NO: 1087 - DNA, 18 bp, CNAG_00031 diagnostic screening primer, pairing with B79
ccgtgttcgcaatctatg

SEQ ID NO: 1088 - DNA, 19 bp, CNAG_00031 Southern blot probe primer
gaatcagcatttgggttcg

SEQ ID NO: 1089 - DNA, 20 bp, NAT#116 STM primer
gcacccaagagctccatctc

SEQ ID NO: 1090 - DNA, 24 bp, STM common primer
gcatgccctgcccctaagaattcg

SEQ ID NO: 1091 - DNA, 19 bp, CNAG_07922 5 flanking region primer 1
cctcttccgctattttgtg

SEQ ID NO: 1092 - DNA, 39 bp, CNAG_07922 5 flanking region primer 2
gctcactggccgtcgttttaccattgctgttgtgggaac

SEQ ID NO: 1093 - DNA, 41 bp, CNAG_07922 3 flanking region primer 1
catggtcatagctgtttcctgaagtggagttggaagaggcg

SEQ ID NO: 1094 - DNA, 22 bp, CNAG_07922 3 flanking region primer 2
caactatccaatacctgttccg

SEQ ID NO: 1095 - DNA, 19 bp, CNAG_07922 diagnostic screening primer, pairing with B79
cacggcttgtcttgaagtc

SEQ ID NO: 1096 - DNA, 18 bp, CNAG_07922 Southern blot probe primer
ttgacggttttggcacag

SEQ ID NO: 1097 - DNA, 20 bp, NAT#116 STM primer
gcacccaagagctccatctc

SEQ ID NO: 1098 - DNA, 24 bp, STM common primer
gcatgccctgcccctaagaattcg

SEQ ID NO: 1099 - DNA, 19 bp, CNAG_04841 5 flanking region primer 1
tgaggtgttccgtgtattg

SEQ ID NO: 1100 - DNA, 35 bp, CNAG_04841 5 flanking region primer 2
ctggccgtcgttttacctcttgactggtaatgggg

SEQ ID NO: 1101 - DNA, 35 bp, CNAG_04841 3 flanking region primer 1
gtcatagctgtttcctgattcccaaggtgacgaag

SEQ ID NO: 1102 - DNA, 20 bp, CNAG_04841 3 flanking region primer 2
tctccaataagttcaggcac

SEQ ID NO: 1103 - DNA, 22 bp, CNAG_04841 diagnostic screening primer, pairing with B79
taaagacggaggtgggagtagg

SEQ ID NO: 1104 - DNA, 18 bp, CNAG_04841 Southern blot probe primer
tgagattgggaaagagcg

SEQ ID NO: 1105 - DNA, 24 bp, NAT#119 STM primer
ctccccacataaagagagctaaac

SEQ ID NO: 1106 - DNA, 24 bp, STM common primer
gcatgccctgcccctaagaattcg

SEQ ID NO: 1107 - DNA, 20 bp, CNAG_01948 5 flanking region primer 1
cttggtaaatccgtattccg

SEQ ID NO: 1108 - DNA, 35 bp, CNAG_01948 5 flanking region primer 2
ctggccgtcgttttaccctttcgcttcaacctacg

SEQ ID NO: 1109 - DNA, 35 bp, CNAG_01948 3 flanking region primer 1
gtcatagctgtttcctgtgatttggcgactctgag

SEQ ID NO: 1110 - DNA, 20 bp, CNAG_01948 3 flanking region primer 2
tgtgtttctcatcgtaagcg

SEQ ID NO: 1111 - DNA, 22 bp, CNAG_01948 diagnostic screening primer, pairing with B79
ttgacttcccaggttacactac

SEQ ID NO: 1112 - DNA, 19 bp, CNAG_01948 Southern blot probe primer
cattgggactcttgtaggg

SEQ ID NO: 1113 - DNA, 24 bp, NAT#119 STM primer
ctccccacataaagagagctaaac

SEQ ID NO: 1114 - DNA, 24 bp, STM common primer
gcatgccctgcccctaagaattcg

SEQ ID NO: 1115 - DNA, 19 bp, CNAG_07435 5 flanking region primer 1
caaccttcaaagtcttgcc

SEQ ID NO: 1116 - DNA, 39 bp, CNAG_07435 5 flanking region primer 2
tcactggccgtcgttttacaacgaggagtcatactgtgc

SEQ ID NO: 1117 - DNA, 41 bp, CNAG_07435 3 flanking region primer 1
catggtcatagctgtttcctgaaaggcgtcaaagggcgaag

SEQ ID NO: 1118 - DNA, 20 bp, CNAG_07435 3 flanking region primer 2
ggtttggagcgtattgattg

SEQ ID NO: 1119 - DNA, 19 bp, CNAG_07435 diagnostic screening primer, pairing with B79
aagagcggcattgaatcgg

SEQ ID NO: 1120 - DNA, 20 bp, CNAG_07435 Southern blot probe primer
gcgtcactttggacatactc

SEQ ID NO: 1121 - DNA, 20 bp, NAT#123 STM primer
ctatcgaccaaccaacacag

SEQ ID NO: 1122 - DNA, 24 bp, STM common primer
gcatgccctgcccctaagaattcg

SEQ ID NO: 1123 - DNA, 22 bp, CNAG_00505 5 flanking region primer 1
tttcaggcaccaacaggcacag

SEQ ID NO: 1124 - DNA, 38 bp, CNAG_00505 5 flanking region primer 2
ctggccgtcgttttacttccgatggtgcccttgagtag

SEQ ID NO: 1125 - DNA, 38 bp, CNAG_00505 3 flanking region primer 1
gtcatagctgtttcctgggtcttccaaatgtcacagtc

SEQ ID NO: 1126 - DNA, 19 bp, CNAG_00505 3 flanking region primer 2
aaagaagagacgcctcacg

SEQ ID NO: 1127 - DNA, 20 bp, CNAG_00505 diagnostic screening primer, pairing with B79
tgatagacaccacggcagtc

SEQ ID NO: 1128 - DNA, 20 bp, CNAG_00505 Southern blot probe primer
cgaggattgtcaaatgaagg

SEQ ID NO: 1129 - DNA, 24 bp, NAT#125 STM primer
cgctacagccagcgcgcgcaagcg

SEQ ID NO: 1130 - DNA, 24 bp, STM common primer
gcatgccctgcccctaagaattcg

SEQ ID NO: 1131 - DNA, 18 bp, CNAG_03115 5 flanking region primer 1
cgaaggaagtaaaacggg

SEQ ID NO: 1132 - DNA, 37 bp, CNAG_03115 5 flanking region primer 2
ctggccgtcgttttacaagcactcaccactctcctac

SEQ ID NO: 1133 - DNA, 36 bp, CNAG_03115 3 flanking region primer 1
gtcatagctgtttcctgtgcttggatagacgacgag

SEQ ID NO: 1134 - DNA, 20 bp, CNAG_03115 3 flanking region primer 2
tcaatcaaagcgttcggggg

SEQ ID NO: 1135 - DNA, 20 bp, CNAG_03115 diagnostic screening primer, pairing with B79
aatccgacttctcagccctg

SEQ ID NO: 1136 - DNA, 20 bp, CNAG_03115 Southern blot probe primer
atctgagggaagggctacag

SEQ ID NO: 1137 - DNA, 20 bp, NAT#177 STM primer
caccaactccccatctccat

SEQ ID NO: 1138 - DNA, 24 bp, STM common primer
gcatgccctgcccctaagaattcg

SEQ ID NO: 1139 - DNA, 19 bp, CNAG_04807 5 flanking region primer 1
gcgtttcctcgtgaacttc

SEQ ID NO: 1140 - DNA, 37 bp, CNAG_04807 5 flanking region primer 2
ctggccgtcgttttacggaagaagggttgagacactc

SEQ ID NO: 1141 - DNA, 36 bp, CNAG_04807 3 flanking region primer 1
gtcatagctgtttcctgggcaagcataatggcaaag

SEQ ID NO: 1142 - DNA, 18 bp, CNAG_04807 3 flanking region primer 2
ggatttccgaagccaaac

SEQ ID NO: 1143 - DNA, 19 bp, CNAG_04807 diagnostic screening primer, pairing with B79
tggcacagttcaatgttcc

SEQ ID NO: 1144 - DNA, 18 bp, CNAG_04807 Southern blot probe primer
cgacaatacaaacacgcc

SEQ ID NO: 1145 - DNA, 20 bp, NAT#177 STM primer
caccaactccccatctccat

SEQ ID NO: 1146 - DNA, 24 bp, STM common primer
gcatgccctgcccctaagaattcg

SEQ ID NO: 1147 - DNA, 19 bp, CNAG_02435 5 flanking region primer 1
atcgttagcagggtgagtc

SEQ ID NO: 1148 - DNA, 42 bp, CNAG_02435 5 flanking region primer 2
gctcactggccgtcgttttactcctattcagggactatcacc

SEQ ID NO: 1149 - DNA, 39 bp, CNAG_02435 3 flanking region primer 1
catggtcatagctgtttcctgacctattttccacgcagc

SEQ ID NO: 1150 - DNA, 18 bp, CNAG_02435 3 flanking region primer 2
tcagcctcgcacataatc

SEQ ID NO: 1151 - DNA, 18 bp, CNAG_02435 diagnostic screening primer, pairing with B79
cgagccgaaaagaacaag

SEQ ID NO: 1152 - DNA, 20 bp, CNAG_02435 Southern blot probe primer
gattatctgtttggttcggc

SEQ ID NO: 1153 - DNA, 24 bp, NAT#184 STM primer
atatatggctcgagctagatagag

SEQ ID NO: 1154 - DNA, 24 bp, STM common primer
gcatgccctgcccctaagaattcg

SEQ ID NO: 1155 - DNA, 20 bp, CNAG_02364 5 flanking region primer 1
gaagtcaacaggaagaagcc

SEQ ID NO: 1156 - DNA, 34 bp, CNAG_02364 5 flanking region primer 2
ctggccgtcgttttactttgcgtgaaggtgtagg

SEQ ID NO: 1157 - DNA, 36 bp, CNAG_02364 3 flanking region primer 1
gtcatagctgtttcctgtgctcatcttcacggctac

SEQ ID NO: 1158 - DNA, 19 bp, CNAG_02364 3 flanking region primer 2
cattatccgcctgatgttg

SEQ ID NO: 1159 - DNA, 19 bp, CNAG_02364 diagnostic screening primer, pairing with B79
gcacttccaacaaagccac

SEQ ID NO: 1160 - DNA, 19 bp, CNAG_02364 Southern blot probe primer
gactttttgcgtgaaggtg

SEQ ID NO: 1161 - DNA, 24 bp, NAT#184 STM primer
atatatggctcgagctagatagag

SEQ ID NO: 1162 - DNA, 24 bp, STM common primer
gcatgccctgcccctaagaattcg

SEQ ID NO: 1163 - DNA, 20 bp, CNAG_05420 5 flanking region primer 1
cgcctttgaggtattcactc

SEQ ID NO: 1164 - DNA, 39 bp, CNAG_05420 5 flanking region primer 2
tcactggccgtcgttttacggtgttggtcacgaatctac

SEQ ID NO: 1165 - DNA, 40 bp, CNAG_05420 3 flanking region primer 1
catggtcatagctgtttcctgcggctttacgaaatgagtg

SEQ ID NO: 1166 - DNA, 21 bp, CNAG_05420 3 flanking region primer 2
cctgaaagacatagcgacaag

SEQ ID NO: 1167 - DNA, 19 bp, CNAG_05420 diagnostic screening primer, pairing with B79
atcctgtcttgctgtggtc

SEQ ID NO: 1168 - DNA, 18 bp, CNAG_05420 Southern blot probe primer
tccagcatcgtcattgag

SEQ ID NO: 1169 - DNA, 20 bp, NAT#191 STM primer
atatggatgtttttagcgag

SEQ ID NO: 1170 - DNA, 24 bp, STM common primer
gcatgccctgcccctaagaattcg

SEQ ID NO: 1171 - DNA, 19 bp, CNAG_05093 5 flanking region primer 1
aatgtattgccaccgtgcc

SEQ ID NO: 1172 - DNA, 41 bp, CNAG_05093 5 flanking region primer 2
tcactggccgtcgttttacttggggtgatgtgttctcgtcc

SEQ ID NO: 1173 - DNA, 41 bp, CNAG_05093 3 flanking region primer 1
catggtcatagctgtttcctgacaggcagattgggaagtgc

SEQ ID NO: 1174 - DNA, 19 bp, CNAG_05093 3 flanking region primer 2
tgtatgccgtgggaacaag

SEQ ID NO: 1175 - DNA, 24 bp, CNAG_05093 diagnostic screening primer, pairing with B79
cgaagtctcaaacctatctactcg

SEQ ID NO: 1176 - DNA, 22 bp, CNAG_05093 Southern blot probe primer
ttgctgaggcgaacttgttggc

SEQ ID NO: 1177 - DNA, 24 bp, NAT#201 STM primer
caccctctatctcgagaaagctcc

SEQ ID NO: 1178 - DNA, 24 bp, STM common primer
gcatgccctgcccctaagaattcg

SEQ ID NO: 1179 - DNA, 19 bp, CNAG_06814 5 flanking region primer 1
tgggaatggcaaaaggcac

SEQ ID NO: 1180 - DNA, 35 bp, CNAG_06814 5 flanking region primer 2
ctggccgtcgttttacggtattttcgtccagtaaa

SEQ ID NO: 1181 - DNA, 35 bp, CNAG_06814 3 flanking region primer 1
gtcatagctgtttcctgtgcagcctatgcctcctt

SEQ ID NO: 1182 - DNA, 19 bp, CNAG_06814 3 flanking region primer 2
taagtgtgttcacggtgcg

SEQ ID NO: 1183 - DNA, 19 bp, CNAG_06814 diagnostic screening primer, pairing with B79
tggttaccgaagtagggag

SEQ ID NO: 1184 - DNA, 19 bp, CNAG_06814 Southern blot probe primer
atttggaggtggagttctg

SEQ ID NO: 1185 - DNA, 22 bp, NAT#208 STM primer
tggtcgcgggagatcgtggttt

SEQ ID NO: 1186 - DNA, 24 bp, STM common primer
gcatgccctgcccctaagaattcg

SEQ ID NO: 1187 - DNA, 21 bp, CNAG_05431 5 flanking region primer 1
catcagtcttgcttcttctgc

SEQ ID NO: 1188 - DNA, 40 bp, CNAG_05431 5 flanking region primer 2
tcactggccgtcgttttacagagtcagaataggtgttggg

SEQ ID NO: 1189 - DNA, 40 bp, CNAG_05431 3 flanking region primer 1
catggtcatagctgtttcctgagggagaggattgaagtgg

SEQ ID NO: 1190 - DNA, 20 bp, CNAG_05431 3 flanking region primer 2
cattactttgactgggaggg

SEQ ID NO: 1191 - DNA, 19 bp, CNAG_05431 diagnostic screening primer, pairing with B79
cacggcaacttatgctctc

SEQ ID NO: 1192 - DNA, 20 bp, CNAG_05431 Southern blot probe primer
actcggtgttggtgaaacgg

SEQ ID NO: 1193 - DNA, 22 bp, NAT#208 STM primer
tggtcgcgggagatcgtggttt

SEQ ID NO: 1194 - DNA, 24 bp, STM common primer
gcatgccctgcccctaagaattcg

SEQ ID NO: 1195 - DNA, 20 bp, CNAG_05642 5 flanking region primer 1
agagggataagagcctgacg

SEQ ID NO: 1196 - DNA, 38 bp, CNAG_05642 5 flanking region primer 2
tcactggccgtcgttttacagaaggaagttgggaagcg

SEQ ID NO: 1197 - DNA, 41 bp, CNAG_05642 3 flanking region primer 1
catggtcatagctgtttcctgatgattacagaggggaggac

SEQ ID NO: 1198 - DNA, 19 bp, CNAG_05642 3 flanking region primer 2
tgtatcccaagcagcaaag

SEQ ID NO: 1199 - DNA, 20 bp, CNAG_05642 diagnostic screening primer, pairing with B79
ctcggaaataaatgtggagc

SEQ ID NO: 1200 - DNA, 20 bp, CNAG_05642 Southern blot probe primer
tacctgccagtgcttcaacc

SEQ ID NO: 1201 - DNA, 20 bp, NAT#210 STM primer
ctagagcccgccacaacgct

SEQ ID NO: 1202 - DNA, 24 bp, STM common primer
gcatgccctgcccctaagaattcg

SEQ ID NO: 1203 - DNA, 19 bp, CNAG_03212 5 flanking region primer 1
gacacccaaacaagcaaac

SEQ ID NO: 1204 - DNA, 39 bp, CNAG_03212 5 flanking region primer 2
gctcactggccgtcgttttacctggggtgtttgttttcg

SEQ ID NO: 1205 - DNA, 41 bp, CNAG_03212 3 flanking region primer 1
catggtcatagctgtttcctggggttcagattttggatacc

SEQ ID NO: 1206 - DNA, 19 bp, CNAG_03212 3 flanking region primer 2
ggcgaggtgttgtaaatcc

SEQ ID NO: 1207 - DNA, 22 bp, CNAG_03212 diagnostic screening primer, pairing with B79
gcgtatctggcatcttgttatc

SEQ ID NO: 1208 - DNA, 18 bp, CNAG_03212 Southern blot probe primer
tgaggaatgccaatggtg

SEQ ID NO: 1209 - DNA, 20 bp, NAT#211 STM primer
gcggtcgctttatagcgatt

SEQ ID NO: 1210 - DNA, 24 bp, STM common primer
gcatgccctgcccctaagaattcg

SEQ ID NO: 1211 - DNA, 18 bp, CNAG_03212 5 flanking region primer 1
gcgaaactttgtgagtgc

SEQ ID NO: 1212 - DNA, 40 bp, CNAG_03212 5 flanking region primer 2
gctcactggccgtcgttttaccaagcagcaagatggagtc

SEQ ID NO: 1213 - DNA, 40 bp, CNAG_03212 3 flanking region primer 1
catggtcatagctgtttcctgtcgtaagttcggtgtcagc

SEQ ID NO: 1214 - DNA, 20 bp, CNAG_03212 3 flanking region primer 2
aagtcttattatgggcgagg

SEQ ID NO: 1215 - DNA, 19 bp, CNAG_03212 diagnostic screening primer, pairing with B79
tgtcccgttgataggtgtc

SEQ ID NO: 1216 - DNA, 20 bp, CNAG_03212 Southern blot probe primer
tcctctccctcctattcagg

SEQ ID NO: 1217 - DNA, 20 bp, NAT#211 STM primer
gcggtcgctttatagcgatt

SEQ ID NO: 1218 - DNA, 24 bp, STM common primer
gcatgccctgcccctaagaattcg

SEQ ID NO: 1219 - DNA, 19 bp, CNAG_07924 5 flanking region primer 1
acctaatcaggaaagcccc

SEQ ID NO: 1220 - DNA, 39 bp, CNAG_07924 5 flanking region primer 2
tcactggccgtcgttttaccattccttctccgaaatctc

SEQ ID NO: 1221 - DNA, 40 bp, CNAG_07924 3 flanking region primer 1
catggtcatagctgtttcctgttatcctcccgaataccgc

SEQ ID NO: 1222 - DNA, 18 bp, CNAG_07924 3 flanking region primer 2
ccgcaccaaactatttcg

SEQ ID NO: 1223 - DNA, 18 bp, CNAG_07924 diagnostic screening primer, pairing with B79
atcgcacgaaaggcaaag

SEQ ID NO: 1224 - DNA, 20 bp, CNAG_07924 Southern blot probe primer
tctaaacccgtctctgactg

SEQ ID NO: 1225 - DNA, 20 bp, NAT#218 STM primer
ctccacatccatcgctccaa

SEQ ID NO: 1226 - DNA, 24 bp, STM common primer
gcatgccctgcccctaagaattcg

SEQ ID NO: 1227 - DNA, 22 bp, CNAG_00156 5 flanking region primer 1
cccgattttgctttttagtgcg

SEQ ID NO: 1228 - DNA, 36 bp, CNAG_00156 5 flanking region primer 2
ctggccgtcgttttacttgccgtctttgcttgggtc

SEQ ID NO: 1229 - DNA, 36 bp, CNAG_00156 3 flanking region primer 1
gtcatagctgtttcctgatcaagtccactcccgaag

SEQ ID NO: 1230 - DNA, 19 bp, CNAG_00156 3 flanking region primer
tagatgatgagggcgaacg

SEQ ID NO: 1231 - DNA, 20 bp, CNAG_00156 diagnostic screening primer, pairing with B79
gcttcgttggttcgttagtc

SEQ ID NO: 1232 - DNA, 20 bp, CNAG_00156 Southern blot probe primer
caatccgtttctctcacctc

SEQ ID NO: 1233 - DNA, 20 bp, NAT#231 STM primer
gagagatcccaacatcacgc

SEQ ID NO: 1234 - DNA, 24 bp, STM common primer
gcatgccctgcccctaagaattcg

SEQ ID NO: 1235 - DNA, 19 bp, CNAG_01173 5 flanking region primer 1
agtatcccaagcatccctc

SEQ ID NO: 1236 - DNA, 39 bp, CNAG_01173 5 flanking region primer 2
tcactggccgtcgttttacggcaggagcaaagtgtattc

SEQ ID NO: 1237 - DNA, 39 bp, CNAG_01173 3 flanking region primer 1
catggtcatagctgtttcctgtatggtggcatctgaacc

SEQ ID NO: 1238 - DNA, 20 bp, CNAG_01173 3 flanking region primer 2
ctgacaagtttaccaggacg

SEQ ID NO: 1239 - DNA, 20 bp, CNAG_01173 diagnostic screening primer, pairing with B79
gcttctgtgtgtctcctctg

SEQ ID NO: 1240 - DNA, 20 bp, CNAG_01173 Southern blot probe primer
gagaaagaaggattccgaag

SEQ ID NO: 1241 - DNA, 24 bp, NAT#242 STM primer
gtagcgataggggtgtcgctttag

SEQ ID NO: 1242 - DNA, 24 bp, STM common primer
gcatgccctgcccctaagaattcg

SEQ ID NO: 1243 - DNA, 19 bp, CNAG_06871 5 flanking region primer 1
tcaggatgggagtgtttgc

SEQ ID NO: 1244 - DNA, 37 bp, CNAG_06871 5 flanking region primer 2
tcactggccgtcgttttacccttctccttttgcttgg

SEQ ID NO: 1245 - DNA, 41 bp, CNAG_06871 3 flanking region primer 1
catggtcatagctgtttcctgcgctcttattaccgcttcag

SEQ ID NO: 1246 - DNA, 20 bp, CNAG_06871 3 flanking region primer 2
tcggtatttcagtagggatg

SEQ ID NO: 1247 - DNA, 19 bp, CNAG_06871 diagnostic screening primer, pairing with B79
cgactgctggatgtatgag

SEQ ID NO: 1248 - DNA, 18 bp, CNAG_06871 Southern blot probe primer
cttgactgcctcatctgc

SEQ ID NO: 1249 - DNA, 21 bp, NAT#295 STM primer
acacctacatcaaaccctccc

SEQ ID NO: 1250 - DNA, 24 bp, STM common primer
gcatgccctgcccctaagaattcg

SEQ ID NO: 1251 - DNA, 18 bp, CNAG_04774 5 flanking region primer 1
atttgaatagccgcaccc

SEQ ID NO: 1252 - DNA, 35 bp, CNAG_04774 5 flanking region primer 2
ctggccgtcgttttacattgggggatgctggaaag

SEQ ID NO: 1253 - DNA, 36 bp, CNAG_04774 3 flanking region primer 1
gtcatagctgtttcctgggtggactgccaaactatg

SEQ ID NO: 1254 - DNA, 19 bp, CNAG_04774 3 flanking region primer 2
aggcatttctgttcctccg

SEQ ID NO: 1255 - DNA, 19 bp, CNAG_04774 diagnostic screening primer, pairing with B79
cgatagacggaggatgaag

SEQ ID NO: 1256 - DNA, 18 bp, CNAG_04774 Southern blot probe primer
atcgttgcttccgcttag

SEQ ID NO: 1257 - DNA, 21 bp, NAT#146 STM primer
actagccccccctcaccacct

SEQ ID NO: 1258 - DNA, 24 bp, STM common primer
gcatgccctgcccctaagaattcg

SEQ ID NO: 1259 - DNA, 18 bp, CNAG_00841 5 flanking region primer 1
tcggcaagtttagcaagc

SEQ ID NO: 1260 - DNA, 39 bp, CNAG_00841 5 flanking region primer 2
gctcactggccgtcgttttacttatttctgggctgtcgc

SEQ ID NO: 1261 - DNA, 40 bp, CNAG_00841 3 flanking region primer 1
catggtcatagctgtttcctgtctgtggagtcagccaaac

SEQ ID NO: 1262 - DNA, 23 bp, CNAG_00841 3 flanking region primer 2
cggtatcctcgtgagtctatttc

SEQ ID NO: 1263 - DNA, 21 bp, CNAG_00841 diagnostic screening primer, pairing with B79
gcagttgctgaagtgaaagac

SEQ ID NO: 1264 - DNA, 20 bp, CNAG_00841 Southern blot probe primer
tgggatagaagaaggctgtg

SEQ ID NO: 1265 - DNA, 24 bp, NAT#205 STM primer
tatccccctctccgctctctagca

SEQ ID NO: 1266 - DNA, 24 bp, STM common primer
gcatgccctgcccctaagaattcg

SEQ ID NO: 1267 - DNA, 18 bp, CNAG_04836 5 flanking region primer 1
tagaaaagccacaacccc

SEQ ID NO: 1268 - DNA, 37 bp, CNAG_04836 5 flanking region primer 2
tcactggccgtcgttttacgagtttcttttggggtgg

SEQ ID NO: 1269 - DNA, 40 bp, CNAG_04836 3 flanking region primer 1
catggtcatagctgtttcctgacgagaaggggaatgatgg

SEQ ID NO: 1270 - DNA, 19 bp, CNAG_04836 3 flanking region primer 2
tgggcatcttgctcattac

SEQ ID NO: 1271 - DNA, 19 bp, CNAG_04836 diagnostic screening primer, pairing with B79
cggagagcaaatagcacag

SEQ ID NO: 1272 - DNA, 20 bp, CNAG_04836 Southern blot probe primer
aggtgtcgtatcgtatttgc

SEQ ID NO: 1273 - DNA, 20 bp, NAT#123 STM primer
ctatcgaccaaccaacacag

SEQ ID NO: 1274 - DNA, 24 bp, STM common primer
gcatgccctgcccctaagaattcg

SEQ ID NO: 1275 - DNA, 19 bp, CNAG_02603 5 flanking region primer 1
tcaaaacgcctttcggaac

SEQ ID NO: 1276 - DNA, 40 bp, CNAG_02603 5 flanking region primer 2
gctcactggccgtcgttttacacaaatggcagttccctcg

SEQ ID NO: 1277 - DNA, 43 bp, CNAG_02603 3 flanking region primer 1
catggtcatagctgtttcctgatctctccctcacttcagtcgg

SEQ ID NO: 1278 - DNA, 19 bp, CNAG_02603 3 flanking region primer 2
taggaccaacttcagaccg

SEQ ID NO: 1279 - DNA, 20 bp, CNAG_02603 diagnostic screening primer, pairing with B79
gcctatggaagaagacaacg

SEQ ID NO: 1280 - DNA, 20 bp, CNAG_02603 Southern blot probe primer
gtcgtgtagttttgaatggc

SEQ ID NO: 1281 - DNA, 19 bp, NAT#224 STM primer
aacctttaaatgggtagag

SEQ ID NO: 1282 - DNA, 24 bp, STM common primer
gcatgccctgcccctaagaattcg

SEQ ID NO: 1283 - DNA, 20 bp, CNAG_03059 5 flanking region primer 1
aatggcgttaccgacgagag

SEQ ID NO: 1284 - DNA, 36 bp, CNAG_03059 5 flanking region primer 2
ctggccgtcgttttacggtattgagagtgccgagtg

SEQ ID NO: 1285 - DNA, 38 bp, CNAG_03059 3 flanking region primer 1
gtcatagctgtttcctgcagactccctcttcttacctg

SEQ ID NO: 1286 - DNA, 24 bp, CNAG_03059 3 flanking region primer 2
cgttactgcgaggttattactgtg

SEQ ID NO: 1287 - DNA, 19 bp, CNAG_03059 diagnostic screening primer, pairing with B79
aaagactcacccttcaacg

SEQ ID NO: 1288 - DNA, 20 bp, CNAG_03059 Southern blot probe primer
cttttttccgctggtttctc

SEQ ID NO: 1289 - DNA, 18 bp, NAT#232 STM primer
ctttaaaggtggtttgtg

SEQ ID NO: 1290 - DNA, 24 bp, STM common primer
gcatgccctgcccctaagaattcg

SEQ ID NO: 1291 - DNA, 21 bp, CNAG_00883 5 flanking region primer 1
cgacagaaacaagtccaagtg

SEQ ID NO: 1292 - DNA, 36 bp, CNAG_00883 5 flanking region primer 2
ctggccgtcgttttacgtagtgaaatgaggattgcg

SEQ ID NO: 1293 - DNA, 35 bp, CNAG_00883 3 flanking region primer 1
gtcatagctgtttcctgtacctgcttttcttgcgg

SEQ ID NO: 1294 - DNA, 18 bp, CNAG_00883 3 flanking region primer 2
acaagcccgaatctcaag

SEQ ID NO: 1295 - DNA, 19 bp, CNAG_00883 diagnostic screening primer, pairing with B79
cttttcactcaatgtcccg

SEQ ID NO: 1296 - DNA, 19 bp, CNAG_00883 Southern blot probe primer
taagaactgttgccctgcc

SEQ ID NO: 1297 - DNA, 18 bp, CNAG_01551 5 flanking region primer 1
tccgttgagatagcgttg

SEQ ID NO: 1298 - DNA, 39 bp, CNAG_01551 5 flanking region primer 2
tcactggccgtcgttttacatggtggaggtgtaggactg

SEQ ID NO: 1299 - DNA, 39 bp, CNAG_01551 3 flanking region primer 1
catggtcatagctgtttcctgttattccccctcaagagc

SEQ ID NO: 1300 - DNA, 20 bp, CNAG_01551 3 flanking region primer 2
gcggcccattcttcttgtcg

SEQ ID NO: 1301 - DNA, 18 bp, CNAG_01551 diagnostic screening primer, pairing with B79
aaccttgcctaacaaccc

SEQ ID NO: 1302 - DNA, 20 bp, CNAG_01551 Southern blot probe primer
ggagtatggctgaaatctgg

SEQ ID NO: 1303 - DNA, 24 bp, NAT#273 STM primer
gagatctttcgggaggtctggatt

SEQ ID NO: 1304 - DNA, 24 bp, STM common primer
gcatgccctgcccctaagaattcg

SEQ ID NO: 1305 - DNA, 20 bp, CNAG_04353 5 flanking region primer 1
tgcgagagagaatgggagac

SEQ ID NO: 1306 - DNA, 38 bp, CNAG_04353 5 flanking region primer 2
tcactggccgtcgttttacggttccatagcgacatcag

SEQ ID NO: 1307 - DNA, 41 bp, CNAG_04353 3 flanking region primer 1
catggtcatagctgtttcctgcgaaggttgtttgtgatacg

SEQ ID NO: 1308 - DNA, 20 bp, CNAG_04353 3 flanking region primer 2
cccaacaactcatcaatctc

SEQ ID NO: 1309 - DNA, 18 bp, CNAG_04353 diagnostic screening primer, pairing with B79
gcattatcgtttcccgac

SEQ ID NO: 1310 - DNA, 22 bp, CNAG_04353 Southern blot probe primer
ttgaggtaggtggagtgttgcc

SEQ ID NO: 1311 - DNA, 20 bp, CNAG_03346 5 flanking region primer 1
cgccctttctattgttacac

SEQ ID NO: 1312 - DNA, 39 bp, CNAG_03346 5 flanking region primer 2
tcactggccgtcgttttacgatgacaggagggatgaatc

SEQ ID NO: 1313 - DNA, 43 bp, CNAG_03346 3 flanking region primer 1
catggtcatagctgtttcctggggagaataacgactcaatgtc

SEQ ID NO: 1314 - DNA, 18 bp, CNAG_03346 3 flanking region primer 2
tcattgctgactgggaag

SEQ ID NO: 1315 - DNA, 18 bp, CNAG_03346 diagnostic screening primer, pairing with B79
aaagaggcggtgttgaag

SEQ ID NO: 1316 - DNA, 19 bp, CNAG_03346 Southern blot probe primer
agccaggtaatcttggagg

SEQ ID NO: 1317 - DNA, 21 bp, NAT#295 STM primer
acacctacatcaaaccctccc

SEQ ID NO: 1318 - DNA, 24 bp, STM common primer
gcatgccctgcccctaagaattcg

SEQ ID NO: 1319 - DNA, 18 bp, CNAG_00239 5 flanking region primer 1
aggattatcgcctgaacc

SEQ ID NO: 1320 - DNA, 37 bp, CNAG_00239 5 flanking region primer 2
tcactggccgtcgttttacatgttgttgaagagggcg

SEQ ID NO: 1321 - DNA, 41 bp, CNAG_00239 3 flanking region primer 1
catggtcatagctgtttcctgaacgacgaccatcgcagtag

SEQ ID NO: 1322 - DNA, 18 bp, CNAG_00239 3 flanking region primer 2
catcccgagttggaaaac

SEQ ID NO: 1323 - DNA, 20 bp, CNAG_00239 diagnostic screening primer, pairing with B79
cactggcgaagtcaagtatg

SEQ ID NO: 1324 - DNA, 20 bp, CNAG_00239 Southern blot probe primer
ctactctgtggtggcgtaag

SEQ ID NO: 1325 - DNA, 20 bp, NAT#296 STM primer
cgcccgccctcactatccac

SEQ ID NO: 1326 - DNA, 24 bp, STM common primer
gcatgccctgcccctaagaattcg

SEQ ID NO: 1327 - DNA, 19 bp, CNAG_03129 5 flanking region primer 1
gcaggcgaaaactattagg

SEQ ID NO: 1328 - DNA, 41 bp, CNAG_03129 5 flanking region primer 2
gctcactggccgtcgttttacgtggggaagtcctcaaatac

SEQ ID NO: 1329 - DNA, 42 bp, CNAG_03129 3 flanking region primer 1
catggtcatagctgtttcctgcgacgacatctcaagtcagag

SEQ ID NO: 1330 - DNA, 20 bp, CNAG_03129 3 flanking region primer 2
tgatgggacgataaaggttc

SEQ ID NO: 1331 - DNA, 19 bp, CNAG_03129 diagnostic screening primer, pairing with B79
tgctttctctaatagcggc

SEQ ID NO: 1332 - DNA, 19 bp, CNAG_03129 Southern blot probe primer
gtgcttttgaagttccgtc

SEQ ID NO: 1333 - DNA, 18 bp, CNAG_03826 5 flanking region primer 1
aatgctgatttggcaggg

SEQ ID NO: 1334 - DNA, 39 bp, CNAG_03826 5 flanking region primer 2
tcactggccgtcgttttaccgatggaagatgttgtcagc

SEQ ID NO: 1335 - DNA, 39 bp, CNAG_03826 3 flanking region primer 1
catggtcatagctgtttcctgacaaagcgaaaggcagac

SEQ ID NO: 1336 - DNA, 18 bp, CNAG_03826 3 flanking region primer 2
cgaaagtgatgcttcagc

SEQ ID NO: 1337 - DNA, 20 bp, CNAG_03826 diagnostic screening primer, pairing with B79
ggaaggtcaggtcctatttg

SEQ ID NO: 1338 - DNA, 20 bp, CNAG_02671 5 flanking region primer 1
cgccgagttatctgacaaag

SEQ ID NO: 1339 - DNA, 41 bp, CNAG_02671 5 flanking region primer 2
tcactggccgtcgttttacttctccaaacaccgcccttgac

SEQ ID NO: 1340 - DNA, 40 bp, CNAG_02671 3 flanking region primer 1
catggtcatagctgtttcctgtaacggggcttagaagtgc

SEQ ID NO: 1341 - DNA, 18 bp, CNAG_02671 3 flanking region primer 2
ttcatcaaaggtctggcg

SEQ ID NO: 1342 - DNA, 20 bp, CNAG_02671 diagnostic screening primer, pairing with B79
cctgactcatcggcttactc

SEQ ID NO: 1343 - DNA, 18 bp, CNAG_02671 Southern blot probe primer
actcctgcttgcgttttc

SEQ ID NO: 1344 - DNA, 20 bp, CNAG_02134 5 flanking region primer 1
ggggtaactatcatcatccg

SEQ ID NO: 1345 - DNA, 38 bp, CNAG_02134 5 flanking region primer 2
tcactggccgtcgttttactctcgctccttttccttcc

SEQ ID NO: 1346 - DNA, 42 bp, CNAG_02134 3 flanking region primer 1
catggtcatagctgtttcctggcagtagaaggtgatacaacg

SEQ ID NO: 1347 - DNA, 19 bp, CNAG_02134 3 flanking region primer 2
cgttacggttggacaatgg

SEQ ID NO: 1348 - DNA, 19 bp, CNAG_02134 diagnostic screening primer, pairing with B79
cgtagaaacaacgcacgag

SEQ ID NO: 1349 - DNA, 21 bp, CNAG_02134 Southern blot probe primer
caagtattctccagggttcag

SEQ ID NO: 1350 - DNA, 20 bp, CNAG_02936 5 flanking region primer 1
gcgagtgatgacgagagttc

SEQ ID NO: 1351 - DNA, 39 bp, CNAG_02936 5 flanking region primer 2
tcactggccgtcgttttacgccttgaccgtctcttctac

SEQ ID NO: 1352 - DNA, 42 bp, CNAG_02936 3 flanking region primer 1
catggtcatagctgtttcctggtctactcgtcactttcatcg

SEQ ID NO: 1353 - DNA, 21 bp, CNAG_02936 3 flanking region primer 2
cgtcacaacaagcactctcac

SEQ ID NO: 1354 - DNA, 19 bp, CNAG_02936 diagnostic screening primer, pairing with B79
ggatgttcaggtgccaatc

SEQ ID NO: 1355 - DNA, 18 bp, CNAG_07460 5 flanking region primer 1
tcggcattggcatacttg

SEQ ID NO: 1356 - DNA, 39 bp, CNAG_07460 5 flanking region primer 2
gctcactggccgtcgttttacgtgatttgagcggtgaag

SEQ ID NO: 1357 - DNA, 42 bp, CNAG_07460 3 flanking region primer 1
catggtcatagctgtttcctgccaaagtggactcaaataggg

SEQ ID NO: 1358 - DNA, 22 bp, CNAG_07460 3 flanking region primer 2
ccgttactttccaaatcaggag

SEQ ID NO: 1359 - DNA, 20 bp, CNAG_07460 diagnostic screening primer, pairing with B79
cgtctgaacctgattctgag

SEQ ID NO: 1360 - DNA, 19 bp, CNAG_07460 Southern blot probe primer
ccgatgaccaaaagtaggc

SEQ ID NO: 1361 - DNA, 19 bp, CNAG_07460 Southern blot probe primer
cagagttgattgccgaaag

SEQ ID NO: 1362 - DNA, 19 bp, CNAG_05436 5 flanking region primer 1
gcccttttgctttaccttc

SEQ ID NO: 1363 - DNA, 41 bp, CNAG_05436 5 flanking region primer 2
tcactggccgtcgttttaccgtagagggatgattttgagac

SEQ ID NO: 1364 - DNA, 40 bp, CNAG_05436 3 flanking region primer 1
catggtcatagctgtttcctggcatccttcgtgctaacag

SEQ ID NO: 1365 - DNA, 18 bp, CNAG_05436 3 flanking region primer 2
gccttgaagaacaaacgg

SEQ ID NO: 1366 - DNA, 19 bp, CNAG_05436 diagnostic screening primer, pairing with B79
gggataggaggcattgatg

SEQ ID NO: 1367 - DNA, 20 bp, CNAG_05436 Southern blot probe primer
caccaaagtggatttccttg

SEQ ID NO: 1368 - DNA, 21 bp, CNAG_05436 Southern blot probe primer
ctcggacaaatcactctactg

SEQ ID NO: 1369 - DNA, 21 bp, CNAG_02698 5 flanking region primer 1
ctacagataatgtgctcagcc

SEQ ID NO: 1370 - DNA, 37 bp, CNAG_02698 5 flanking region primer 2
tcactggccgtcgttttactttgttccatagccagcg

SEQ ID NO: 1371 - DNA, 40 bp, CNAG_02698 3 flanking region primer 1
catggtcatagctgtttcctggttctgtcttgaagggtgc

SEQ ID NO: 1372 - DNA, 20 bp, CNAG_02698 3 flanking region primer 2
cggtgaagttggctaagaac

SEQ ID NO: 1373 - DNA, 19 bp, CNAG_02698 diagnostic screening primer, pairing with B79
gaaagggctaagaagcgac

SEQ ID NO: 1374 - DNA, 20 bp, CNAG_02698 Southern blot probe primer
aaactctccatctgtgtccc

SEQ ID NO: 1375 - DNA, 20 bp, CNAG_04600 5 flanking region primer 1
gctgttggctgattgtttac

SEQ ID NO: 1376 - DNA, 39 bp, CNAG_04600 5 flanking region primer 2
tcactggccgtcgttttacttacagtatcccaccgtccc

SEQ ID NO: 1377 - DNA, 40 bp, CNAG_04600 3 flanking region primer 1
catggtcatagctgtttcctgtgggagtgatgtctttggc

SEQ ID NO: 1378 - DNA, 18 bp, CNAG_04600 3 flanking region primer 2
ccctcaaaagttgcgaag

SEQ ID NO: 1379 - DNA, 18 bp, CNAG_04600 diagnostic screening primer, pairing with B79
ctggattttggaatgggc

SEQ ID NO: 1380 - DNA, 18 bp, CNAG_04600 Southern blot probe primer
ttacatttgccagcggac